European Patent Application EP 4 603 579 A2, published August 20, 2025. Title: ENGINEERED PRODUCER CELL LINES AND METHODS OF MAKING AND USING THE SAME. Applicant: ULTRAGENYX PHARMACEUTICAL INC. Application EP. The sequence listing filed with the application follows.

SEQUENCE LISTING (59 sequences)

SEQ ID NO: 1 - RNA, 21 nt, synthetic construct
  source 1..21: mol_type = other RNA
gcaacagcgtaaaaattgttt

SEQ ID NO: 2 - RNA, 21 nt, synthetic construct
  source 1..21: mol_type = other RNA
cggtgtccacagtccttgatt

SEQ ID NO: 3 - RNA, 21 nt, synthetic construct
  source 1..21: mol_type = other RNA
caagaaaagttataagttttt

SEQ ID NO: 4 - RNA, 21 nt, synthetic construct
  source 1..21: mol_type = other RNA
cggaggaagttacagatgttt

SEQ ID NO: 5 - RNA, 21 nt, synthetic construct
  source 1..21: mol_type = other RNA
agatgcaagaggtaccaaatt

SEQ ID NO: 6 - RNA, 21 nt, synthetic construct
  source 1..21: mol_type = other RNA
ggtgtcggatgatttatcatt

SEQ ID NO: 7 - RNA, 21 nt, synthetic construct
  source 1..21: mol_type = other RNA
gaagctagaacttaccaaatt

SEQ ID NO: 8 - RNA, 21 nt, synthetic construct
  source 1..21: mol_type = other RNA
ggatgtctttcctaggagatt

SEQ ID NO: 9 - RNA, 21 nt, synthetic construct
  source 1..21: mol_type = other RNA
cgctcatcgacaataattatt

SEQ ID NO: 10 - RNA, 21 nt, synthetic construct
  source 1..21: mol_type = other RNA
cactttagatgtatctaattt

SEQ ID NO: 11 - RNA, 21 nt, synthetic construct
  source 1..21: mol_type = other RNA
ggagcataaagtagaccgatt

SEQ ID NO: 12 - RNA, 20 nt, synthetic construct
  source 1..20: mol_type = other RNA
ttgccactacagctaccacc

SEQ ID NO: 13 - RNA, 20 nt, synthetic construct
  source 1..20: mol_type = other RNA
ccaatgtactcagggaaaca

SEQ ID NO: 14 - RNA, 20 nt, synthetic construct
  source 1..20: mol_type = other RNA
agtccaccaaagtgtttgct

SEQ ID NO: 15 - RNA, 20 nt, synthetic construct
  source 1..20: mol_type = other RNA
aaaggagtctgcttacttac

SEQ ID NO: 16 - DNA, 20 bp, Homo sapiens
  source 1..20: mol_type = genomic DNA
ttgccactacagctaccacc

SEQ ID NO: 17 - DNA, 20 bp, Homo sapiens
  source 1..20: mol_type = genomic DNA
ccaatgtactcagggaaaca

SEQ ID NO: 18 - DNA, 20 bp, Homo sapiens
  source 1..20: mol_type = genomic DNA
agtccaccaaagtgtttgct

SEQ ID NO: 19 - DNA, 20 bp, Homo sapiens
  source 1..20: mol_type = genomic DNA
aaaggagtctgcttacttac

SEQ ID NO: 20 - DNA, 20 bp, Homo sapiens
  source 1..20: mol_type = genomic DNA
cttctcgtaatggcagatct

SEQ ID NO: 21 - DNA, 20 bp, Homo sapiens
  source 1..20: mol_type = genomic DNA
gcacttgaggatcttgcacg

SEQ ID NO: 22 - DNA, 20 bp, Homo sapiens
  source 1..20: mol_type = genomic DNA
gaggtcctctatgccatgga

SEQ ID NO: 23 - DNA, 20 bp, Homo sapiens
  source 1..20: mol_type = genomic DNA
ccatacccatccatccagct

SEQ ID NO: 24 - DNA, 20 bp, Homo sapiens
  source 1..20: mol_type = genomic DNA
cccatgtgaaggaccttcaa

SEQ ID NO: 25 - DNA, 20 bp, Homo sapiens
  source 1..20: mol_type = genomic DNA
gttcttcaaactctgttcgg

SEQ ID NO: 26 - DNA, 20 bp, Homo sapiens
  source 1..20: mol_type = genomic DNA
gaaggcgtagacttatctga

SEQ ID NO: 27 - DNA, 20 bp, Homo sapiens
  source 1..20: mol_type = genomic DNA
agccaacttccagcaccaat

SEQ ID NO: 28 - DNA, 20 bp, Homo sapiens
  source 1..20: mol_type = genomic DNA
gggcaatggaccttctgcct

SEQ ID NO: 29 - DNA, 20 bp, Homo sapiens
  source 1..20: mol_type = genomic DNA
ggctgcggggcagagggcaa

SEQ ID NO: 30 - DNA, 20 bp, Homo sapiens
  source 1..20: mol_type = genomic DNA
cgggcaggctgcggggcaga

SEQ ID NO: 31 - DNA, 20 bp, Homo sapiens
  source 1..20: mol_type = genomic DNA
acgggcaggctgcggggcag

SEQ ID NO: 32 - RNA, 21 nt, synthetic construct
  source 1..21: mol_type = other RNA
acaatttttacgctgttgcca

SEQ ID NO: 33 - RNA, 21 nt, synthetic construct
  source 1..21: mol_type = other RNA
tcaaggactgtggacaccggt

SEQ ID NO: 34 - RNA, 21 nt, synthetic construct
  source 1..21: mol_type = other RNA
aaacttataacttttcttgga

SEQ ID NO: 35 - RNA, 21 nt, synthetic construct
  source 1..21: mol_type = other RNA
acatctgtaacttcctccgca

SEQ ID NO: 36 - RNA, 21 nt, synthetic construct
  source 1..21: mol_type = other RNA
tttggtacctcttgcatctca

SEQ ID NO: 37 - RNA, 21 nt, synthetic construct
  source 1..21: mol_type = other RNA
tgataaatcatccgacacctg

SEQ ID NO: 38 - RNA, 21 nt, synthetic construct
  source 1..21: mol_type = other RNA
tttggtaagttctagcttcct

SEQ ID NO: 39 - RNA, 21 nt, synthetic construct
  source 1..21: mol_type = other RNA
tctcctaggaaagacatccaa

SEQ ID NO: 40 - RNA, 21 nt, synthetic construct
  source 1..21: mol_type = other RNA
taattattgtcgatgagcggc

SEQ ID NO: 41 - RNA, 21 nt, synthetic construct
  source 1..21: mol_type = other RNA
attagatacatctaaagtggg

SEQ ID NO: 42 - RNA, 21 nt, synthetic construct
  source 1..21: mol_type = other RNA
tcggtctactttatgctcctt

SEQ ID NO: 43 - RNA, 3610 nt, Homo sapiens
  source 1..3610: mol_type = mRNA
cttcctgcggctgaaccgcccggctgagccgacattgccggcgtcttggcgattcggcccgacgagctccgctttcgctacagcatggtggcctactggagacaggctggactcagctacatccgatactcccagatctgtgcaaaagcagtgagagatgcactgaagacagaattcaaagcaaatgctgagaagacttctggcagcaacgtaaaaattgtgaaagtaaagaaggaataatctaccctgactaaagcttgaaatgctacatttccaaggtgaagatgtgtgggcacatgttatggcagattgaaaaggatctcattccatgggaaaaaaaaaaatcctgtcttgttcataaattgacaatgtcaataaattgaaatatggttcactgttactcttgattttagtttgtgagactttttcattttctttaaaggaactgtctgcacagctgcatgattatggccatgtgaaccagggtttcttaaaagcaggggaagccagatttaatatttagtgaccaaagggatacagaaagcattttgaaaatgtctcaaaatagttgtttcatgacattaattggtgatcaaaattatctgctgtcattgaggcttcgtagtcccttatttttgaattgttgtcatgtcagaataatgacatggttatcagtaacaaatggaaataattattaaatactaaaagtgtagattagaagaagaaatactaaattgtacttgttttgtattgtgcacttaaagcctatagataagaacggttacagaatttaagcacaaagtgtttttcacattgttttgtaaatgaatctttatactctggtagcatttctcataggaaatgaggcaaagctattgaataacttgctcattgagttgatggccaaactgaaattaaaacctaggagttttgactgcaagtctgggacacggtgaccacaacagcagtttcgtggtatttccatagtgattcattcattcattatttagggatgaaaaattgttgcaagttatgtttttatctttctttgaaacttgaaagggcttgggcaagtaaaacaccattgcaaagttaactgcctgattttaactgtttttggagactggagaaataaatttgaactggaaattttgaaacaccattctaggatcagttctcacatggtacttaagctcacaatgatttatcagggccactgtcagcaatgccgaggataagccgaaaagaacatctttgttctcggcttctgggaatgacttattgtcccgacacttgacctgtaggttttactgaattctcagcacagagcgagcagggaggcagagccaattgagtggaagagggtgcctctggaaaacagcaggttaggagcccttggagtcctccgcctcggagctgtcatcctgctgttggcaagttagggcacctcagttcagtgctgtggcccccaagattaaggtactaggaagtatcctccattacagggaacaggaataaatgaatcaaaaagctatcgggcctttttgacatgggacgaataaagtaactaataggcaaaggggctaaatgatttccagtcaagtaattagagataagtcatttattaaggaggcagatggggtattattggtatatagatggcatagtagattgctagtatattggtagattattggtatatagatggtatgttaaggaggcagatggggtattactggtatatagatggtatggtagattggtagtatattggcagattattggtatatggtatgttgaggcagatggggtattactggtatatagatggcatagtagattggtagtatattggtagattattggtatagagatggtatattattaaggaggcagatggggtaattagaggtgagacttagggacagggcttgtgatatggaaaggagtgaagtcactgagtaaaagacaagtttactgtcagcagagattcttagaggctcttttctccgtgattaaaaaaaaatcctaaaccagtagtataataaacttcctgcctccagcagtgctgggtagctggcaggatgactgtgcccagtgatgaggtgaccccagtcagaccaacttaatgagtatcccactaattagttggatgatgtttgaagctgtcagttaatctcttagttcacatcgttcttgtgagcaaagtgaaggaatcggataagctctaaatttcggtgatgctgctgctctgagagaccaaggtcgctggagcaaccgtactgctaaaggataagctcttcaaaatcaaaagggacagatttcttaagtttctagtttgttttgtgtttttacatctatttctaccatacgaaagagtaggatggtgagatgcatttctaaatatttttaactactcagtctggatggttaggcttcaagaaaaggaatttatttagtctgaaataaagcaattttgccatttaaaattgaattactttgtagtttaatgattactattgagcaaacaaatctttacagtaatataagtcagcaaaagttttttaaaaggtttaaatccctccttccttacatctatttcattgcttttttaggtttgggaagtaaagcaccagaggaagcatgtgtaaatccttgtataatcgcaggctgtaagtctttagcatctcaggaagttactaacttcaaactaagtatataggtagagtttcttactaaatctagtgcttcttgaaccacaagtagaaagcatttaaaacatgaatgttgttttgtgttttttgaagtttgtaaatagaagacttgttgatgatccgatggcaaggtatttttctcttggtatgtattttagttatttcctcgtgatgcataagtgaaaagagtgaagtttctcagaatgagcaactgtcatccatctacctgctattttattattgctgattacaaaagcaaatcaagagatgagaacccagttgcctgcaagtaaatatttactgcattgagggtcggagcattttcccattaccggttatccatggatcaaatagtgtatctcagtggtaattctagagggccattaaaaccctgatggtgctggaagagatggcagtgctgcatgtcagaaataggtaaactgtaattaagaagttacagatgatttgattacgctcttgtgtatttggtcctgttataatgtgagcagattaaaatcatgtagtgcttaaagctatgtcattatgcaaacatttatggcaacttctgcaaattaatttgaactgtaaaagttccctaatgagacgatgtcctccataactgagaaggacactgcagccattgctgcttaattcctgcatttgaatggttgccgagcgcatggtgtgccctttctcaaagagcagagaggctgcagagcattttggggggtgatgactgaatgaaagtgaaaagaccatttcaaaatagcctttaaaaggaaagccaaggatgattattaatgaattcctgggatctaacagtagtaagaaatttaaactatataaacatatatgttaaaggctagctcttcagaaataaagatcagaagactgca

SEQ ID NO: 44 - DNA, 568 bp, Homo sapiens
  source 1..568: mol_type = genomic DNA
gaacccgggaggtggagggtgcagtgagccaagatcacatcactgcacttcagcctgggcaacaagagtaaaactccgtctaaaaaaaaagaaaaaaaaggacattgccagagtcttggcgatttggcccgacgcgctccgctttcgctacagcatggtggcctactggagacaggctggactcagctacatccgatactcccagatctgtgcaaaagtagtgagagatgcactgaagacagaattcaaagcaaatgccaaaaagacttctggcaacagcgtaaaaattgtgaaagtaaagaaggaataatctaccctgactaaagcttgaaatgctgcatttccaaggtgaagatgtatgggcacatgttatggcagattgaaaaggatctcatttcatgggaaaaaaaaatcctgtcttgttcataaattgacaatgtcaataaattgaaatatggttcactgttaaaaaaaaaaaaaaaaaaggttggaaagtgcaaggcaaggaaatggattctctcccagaaacctccagaaggaaccagccctgccaacaccttgattttag

SEQ ID NO: 45 - RNA, 3013 nt, Homo sapiens
  source 1..3013: mol_type = mRNA
cattgccctctgccccgcagcctgcccgttcccaggccagcgagggcgctcccaggccggtctgcagccagaacacagcccgttccatgtgcttgtcctcgggacacattaggaatgaacccaggcctcagtcctggcctcctcctcaaggctgggtgctcagacgtccccctcagcccctttctctagaccttccggctgaacaaacgagaacatctcacagccctgcaacagccaggagctgctcgtggagctccacgcccggctggagagagaggaggcaccctgggcagcccgccagcacccaggctctcacagtggaagcccacgtcttcttgggctctattttgaaagctgttctttccacgacggctttgacaagaatcgatttgagtgagccggcgtgtcaatacaggccagcacaggactggcctcagggccacattggggagggtggcgaccaggccctggctgcagcccacgtgggcaaaagcatggccaggcaggaggtggggcctgtgagcttggctacagcgaccgtgggcgctgggcccggggctcctcagccctgaggggagacccaggcccaggcaggctcccaggcgggctcccgggctcccagccttccgatcttctccctttgagaccttgccttctgcacagtgacaggaaagagccctgagtcccactttgcagggatgtattgcatttccagaaagttccttccgggtgcagagtgatacatgaaccctggggactcactccaacttggtattgattttctccacggaggacccagcagtcacggcccgtgtctgcacagccccttggatcctgcggaggaattcagccggcccctccccctgtgccgaaaaccacggaggcaaagccaggccagggtacagtgagaacacgggagaggactgagagaccgctggctgccgagggaggaagagcaggattcgcacccccgtcatcgctgggcccacacgccgccgacagcttccgcgtgtggccatctgtctttcagaaactctctggcagagggacccagcagatgacacgggggccgttcacactctgaaacctgcctggagtcaaaacactgctggcgagcctccaccgcaaacccaatccagatggtcttccctggtggccctcggggtggcgggcaccctgcccactccctgccagcccctgcccgctggactccaggcccggtcgagcccccgaccggtctcctgacccagcatgctgctctcccctgggcccggcttcctcgcccgctgggactcccaggcccctccagcccagccccgagagcaggagccccaagggaggcttggcggctgtggaggcgagtgggccacgtgtagctgggaggccggcaggaccaggagcccctcacagcgcagcacccacagcatcacgagccacttccactcctgggtggcctgggggcccccaccctgctctgagctgccccttgttgtgacctggggtcccccgtggtgggcccgccccttgagcctgggatccagcctcagcgaggctccagaagtgtcgtctccgccggccaggcgtcagcgcctccacccaggatcacacactcctatctctgcacttctgccctccatcctgctccacgccgcctctgcttgttattccagcacattccagggtgatgcctgctgaagccacgcagccagtgcctccaccctaccccccatctgacccaccggccccttccgcacgctggaagcctgcccggcctgaagtgtcctcacctgtcgccctatcctcccctccactccagcccaccggtgactcagccctcacagctctctcctccccgagggagccggtgacttggctctgatggtgccgggacccagccccggcatgttcagaatccttgtcctttaacctgcgtccacatgtagtcgcctccacctccctgcctgaacctccaggccctgcagagcaaacactgctgcctgcaggagacccctggggccttctccgtcccctcatcctcctaaggagcctcccctgccaccgtgccagaatgtgccggaggaacagaggcccgagcctcccgtggccccagcgaggcttcctctggggaagacagtgagcccaacgccctggctctcgaggggtggacggagtccagctggcatcaaccgggtgcccctcttcaccggtgtccacagtccttgagagcaaagggttcccagaggcgacctccctcctgcacaggcatttgtcatccttaccctctaggacagctttgccatgtgcagtgaacccctggacagtgttgcgtgccactttgccggatttggactgtatacagaccgaagcatgtggcatgaagccttctgctgtcagcaagttccttgtccctcgacagtatgtgcccaggctgcccttcaaggtggcagtgatggcagttgtctcttgcacgctgcgtacagttctgtcactgactcttacacacagccctggagacgggagagtgccgggagcattctatgcaagtgtcctggcctttgcgggcgtctccacagcacaaacacgagtcagggaccacccctcttctgcttccatgattccaccaactgggtggggcagagcagtgccagggccggaggcacgccccaggtgagggcaggtggccatgccagtgagtgcactgcgttctcagttaattcatccgaaatatttctaagtttcttgattattgcagttgcatccccaagataatgccgccctcaccaagtagaaggcacatgtgctctgatggcccctcccacactggggtcagggcacagcaacttagcgaggcgacgtgggggctcagaggacctcggaccaggctcggcacatggggcttctccagccagccagggggaagcaccctgcagactgctaacttttgcaaaatagagtaaaaaagatcagctagaaaaataaaacaaaaaaggaaagatatacaaaatacaaggcc

SEQ ID NO: 46 - RNA, 3015 nt, Homo sapiens
  source 1..3015: mol_type = unassigned RNA
cattgccctctgccccgcagcctgcccgttcccaggccagcgagggcgctcccaggccggtctgcagccagaacacagcccgttccatgtgcttgtcctcgggacacattaggaatgaacccaggcctcagtcctggcctcctcctcaaggctgggtgctcagacgtccccctcagcccctttctctagaccttccggctgaacaaacgagaacatctcacagccctgcaacagccaggagctgctcgtggagctccacgcccggctggagagagaggaggcaccctgggcagcccgccagcacccaggctctcacagtggaagcccacgtcttcttgggctctattttgaaagctgttctttccacgacggctttgacaagaatcgatttgagtgagccggcgtgtcaatacaggccagcacaggactggcctcagggccacattggggagggtggcgaccaggccctggctgcagcccacgtgggcaaaagcatggccaggcaggaggtggggcctgtgagcttggctacagcgaccgtgggcgctgggcccggggctcctcagccctgaggggagacccaggcccaggcaggctcccaggcgggctcccgggctcccagccttccgatcttctccctttgagaccttgccttctgcacagtgacaggaaagagccctgagtcccactttgcagggatgtattgcatttccagaaagttccttccgggtgcagagtgatacatgaaccctggggactcactccaacttggtattgattttctccacggaggacccagcagtcacggcccgtgtctgcacagccccttggatcctgcggaggaattcagccggcccctccccctgtgccgaaaaccacggaggcaaagccaggccagggtacagtgagaacacgggagaggactgagagaccgctggctgccgagggaggaagagcaggattcgcacccccgtcatcgctgggcccacacgccgccgacagcttccgcgtgtggccatctgtctttcagaaaccctctggcagagggacccagcagatgacacgggggccgttcacactctgaaacctgcctggagtcaaaacactgctggcgagcctccaccgcaaacccaatccagatggtcttccctggtggccctcggggtggcgggcaccctgcccactccctgccagcccctgcccgctggactccaggcccggccgagcccccgaccggtctcctgacccagcatgctgctctcccctgggcccggctttctcgcccgctgggactcccaggcccctccagcccagccccgagagcaggagccccaagggaggcttggcggctgtggaggcgagtgggccacgtgtagctgggaggccggcaggaccaggagcccctcacagcgcagcacccacagcatcacgagccacttccactcctgggtggcctgggggcccccaccctgctctgagctgccccttgttgtgacctggggtcccccgtggtgggcccgccccttgagcctgggatccagcctcagcgaggctccagaagtgtcgtctccgccggccaggcgtcagcgcctccacccaggatcacacactcctatctctgcacttctgccctccatcctgctccacgccgcctctgcttgttattccagcacattccagggtgatgcctgctgaagccacgcagccagtgcctccaccctaccccccatctgacccaccggccccttccgcacgctggaagcctgcccggcctgaagtgtcctcacctgtcgccctatcctcccctccactccagcccaccggtgactcagccctcacagctctctcctccccgagggagccggtgacttggctctgatggtgccgggacccagccccggcatgttcagaatccttgtcctttaacctgcgtccacatgtagtcgcctccacctccctgcctgaacctccaggccctgcagagcaaacactgctgcctgcaggagacccctggggccttctccgtcccctcatcctcctaaggagcctcccctgccaccgtgccagaatgtgccggaggaacagaggcccgagcctcccgtggccccagcgaggcttcctctggggaagacagtgagcccaacgccctggctctcgaggggtggacggagtccagctggcatcgaccgggtgcccctcttcaccggtgtccacagtccttgagagcaaagggttcccagaggcgacctccctcctgcacaggcatttgtcatccttaccctctaggacagctttgccatgtgcagtgaacccctggacagtgttgcgtgccactttgccggatttggactgtatacagaccgaagcatgtggcatgaagccttctgctgtcagcaagttccttgtccctcgacagtatgtgcccaggctgcccttcaaggtggcagtgatggcagttgtctcttgcacgctgcgtacagttctgtcactgactcttacacacagccctggagacgggagagtgccgggagcattctatgcaagtgtcctggcctttgcgggcgtctccacagcacaaacacgagtcagggaccacccctcttctgcttccatgattccaccaactgggtggggcagagcagtgccagggccggaggcacgccccaggtgagggcaggtggccatgccagtgagtgcactgcgttctcagttaattcatccgaaatatttctaagtttcttgattattgcagttgcatccccaagataatgccgccctcaccaagtagaaggcacatgtgctctgatggcccctcccacactggggtcagggcacagcaacttagcgaggcgacgtgggggctcagaggacctcggaccaggctcggcacatggggcttctccagccagccagggggaagcaccctgcagactgctaacttttgcaaaatagagtaaaaaagatcagctagaaaaataaaacaaaaaaggaaagatatacaaaaaaaaaaaaaaa

SEQ ID NO: 47 - RNA, 2079 nt, Homo sapiens
  source 1..2079: mol_type = mRNA
actgctgtgcagggcaggaaagctccacacacacagcccagcaaacagcagcacgctgctgaaaaaaagactcagaggagagagataaggaaggaaagtagtgatggatctcatcccaaacttggccgtggaaacctggcttctcctggctgtcagcctgatactcctctatctatatggaacccgtacacatggactttttaagaagcttggaattccagggcccacacctctgccttttttgggaaatgctttgtccttccgtaagggctattggacgtttgacatggaatgttataaaaagtatagaaaagtctggggtatttatgactgtcaacagcctatgctggctatcacagatcccgacatgatcaaaacagtgctagtgaaagaatgttattctgtcttcacaaaccggaggcctttcgggccagtgggatttatgaaaaatgccatctctatagctgaggatgaagaatggaagagaatacgatcattgctgtctccaacattcaccagcggaaaactcaaggagatggtccctatcattgcccagtatggagatgtgttggtgagaaatctgaggcgggaagcagagacaggcaagcctgtcaccttgaaacacgtctttggggcctacagcatggatgtgatcactagcacatcatttggagtgagcatcgactctctcaacaatccacaagacccctttgtggaaaacaccaagaagcttttaagatttaatccattagatccattcgttctctcaataaaagtctttccattccttaccccaattcttgaagcattaaatatcactgtgtttccaagaaaagttataagttttctaacaaaatctgtaaaacagataaaagaaggtcgcctcaaagagacacaaaagcaccgagtggatttccttcagctgatgattgactctcagaattcaaaagactctgagacccacaaagctctgtctgatctggagctcatggcccaatcaattatctttatttttgctggctatgaaaccacgagcagtgttctctccttcattatatatgaactggccactcaccctgatgtccagcagaaagtgcagaaggaaattgatacagttttacccaataaggcaccacccacctatgatactgtgctacagttggagtatcttgacatggtggtgaatgaaacactcagattattcccagttgctatgagacttgagagggtctgcaaaaaagatgttgaaatcaatgggatgtttattcccaaaggggtggtggtgatgattccaagctatgttcttcatcatgacccaaagtactggacagagcctgagaagttcctccctgaaaggttcagtaaaaagaacaaggacaacatagatccttacatatacacaccctttggaagtggacccagaaactgcattggcatgaggtttgctctcgtgaacatgaaacttgctctagtcagagtccttcagaacttctccttcaaaccttgtaaagaaacacagatccccctgaaattacgctttggaggacttcttctaacagaaaaacccattgttctaaaggctgagtcaagggatgagaccgtaagtggagcctgatttccctaaggacttctggtttgctctttaagaaagctgtgccccagaacaccagagacctcaaattactttacaaatagaaccctgaaatgaagacgggcttcatccaatgtgctgcataaataatcagggattctgtacgtgcattgtgctctctcatggtctgtatagagtgttatacttggtaatatagaggagatgaccaaatcagtgctggggaagtagatttggcttctctgcttctcataggactatctccaccacccccagttagcaccattaactcctcctgagctctgataacataattaacatttctcaataatttcaaccacaatcattaataaaaataggaattattttgatggctctaacagtgacatttatatcatgtgttatatctgtagtattctatagtaagctttatattaagcaaatcaataaaaacctctttacaaaagtat

SEQ ID NO: 48 - RNA, 6348 nt, Homo sapiens
  source 1..6348: mol_type = mRNA
aattaattttacttaggataagtgttgttattattgtttttattgttgttctgttagttactcaaaacttcattctaattgtgccctgagtttgttaaaataccatactgtatttttgtgtaacatgtaaataggcattaatttttgagaaatagaaatgtttatccttaatgtatttttaatttgctaacattgattttttattttctttcctgaaatagcttatttcctaaaatgaaagaatttattctcagatgaataatttttatatcagctattcttatcagagcaataaacaaataccaatgatgcgctcagccaacaattcattacactctctgaagagtaactggacaaggagaaaaacatagggaaaaaaccaacagaatttgttggcatgttctacacacagaccatggcttttcagaagccaagctgaatcaaaacagttttaaaagaggcaaccatttgtagaggagtccttgaaggattcttcattgttttcttggacaaaaagagaccagtggatccaagtgcttcaaatacttctctcttattttcttaactctattgctctgcaatatttactttaccctgttaatgaacaggacaaaatggttaaaaaagagataagcgtgcgtcaacaaattcaggctcttctgtacaagaattttcttaaaaaatggagaataaaaagagagtttattggaatggacaataacattgtttctagggctatatttgtgcatcttttcggaacacttcagagctacccgttttcctgaacaacctcctaaagtcctgggaagcgtggatcagtttaatgactctggcctggtagtggcatatacaccagtcagtaacataacacaaaggataatgaataagatggccttggcttcctttatgaaaggaagaacagtcattgggacaccagatgaagagaccatggatatagaacttccaaaaaaataccatgaaatggtgggagttatatttagtgatactttctcatatcgcctgaagtttaattggggatatagaatcccagttataaaggagcactctgaatacacagaacactgttgggccatgcatggtgaaattttttgttacttggcaaagtactggctaaaagggtttgtagcttttcaagctgcaattaatgctgcaattatagaagtcacaacaaatcattctgtaatggaggagttgacatcagttattggaataaatatgaagataccacctttcatttctaagggagaaattatgaatgaatggtttcattttacttgcttagtttctttctcttcttttatatactttgcatcattaaatgttgcaagggaaagaggaaaatttaagaaactgatgacagtgatgggtctccgagagtcagcattctggctctcctggggattgacatacatttgcttcatcttcattatgtccatttttatggctctggtcataacatcaatcccaattgtatttcatactggcttcatggtgatattcacactctatagcttatatggcctttctttgatagcattggctttcctcatgagtgttttaataaggaaacctatgctcgctggtttggctggatttctcttcactgtattttggggatgtctgggattcactgtgttatatagacaacttcctttatctttgggatgggtattaagtcttcttagcccttttgccttcactgctggaatggcccagattacacacctggataattacttaagtggtgttatttttcctgatccctctggggattcatacaaaatgatagccacttttttcattttggcatttgatactcttttctatttgatattcacattatattttgagcgagttttacctgataaagatggccatggggattctccattatttttccttaagtcctcattttggtccaaacatcaaaatactcatcatgaaatctttgagaatgaaataaatcctgagcattcctctgatgattcttttgaaccggtgtctccagaattccatggaaaagaagccataagaatcagaaatgttataaaagaatataatggaaagactggaaaagtagaagcattgcaaggcatattttttgacatatatgaaggacagatcactgcaatacttgggcataatggagctggtaaatcaacactgctaaacattcttagtggattgtctgtttctacagaaggatcagccactatttataatactcaactctctgaaataactgacatggaagaaattagaaagaatattggattttgtccacagttcaattttcaatttgacttcctcactgtgagagaaaacctcagggtatttgctaaaataaaagggattcagccaaaggaagtggaacaagaggtaaaaagaattataatggaattagacatgcaaagcattcaagacattattgctaaaaaattaagtggtgggcagaagagaaaactaacactagggattgccatcttaggagatcctcaggttttgctgctagatgaaccaactgctggattggatcccttttcaagacaccgagtgtggagcctcctgaaggagcataaagtagaccgacttatcctcttcagtacccaattcatggatgaggctgacatcttggctgataggaaagtatttctgtctaatgggaagttgaaatgtgcaggatcatctttgtttctgaagcgaaagtggggtattggatatcatttaagtttacacaggaatgaaatgtgtgacacagaaaaaatcacatcccttattaagcagcacattcctgatgccaagttaacaacagaaagtgaagaaaaacttgtatatagtttgcctttggaaaaaacgaacaaatttccagatctttacagtgaccttgataagtgttctgaccagggcataaggaattatgctgtttcagtgacatctctgaatgaagtattcttgaacctagaaggaaaatcagcaattgatgaaccagattttgacattgggaaacaagagaaaatacatgtgacaagaaatactggagatgagtctgaaatggaacaggttctttgttctcttcctgaaacaagaaaggctgtcagtagtgcagctctctggagacgacaaatctatgcagtggcaacacttcgcttcttaaagttaaggcgtgaaaggagagctcttttgtgtttgttactagtacttggaattgcttttatccccatcattctagagaagataatgtataaagtaactcgtgaaactcattgttgggagttttcacccagtatgtatttcctttctctggaacaaatcccgaagacgcctcttaccagcctgttaatcgttaataatacaggatcaaatattgaagacctcgtgcattcactgaagtgtcaggatatagttttggaaatagatgactttagaaacagaaatggctcagatgatccctcctacaatggagccatcatagtgtctggtgaccagaaggattacagattttctgttgcgtgtaataccaagaaattgaattgttttcctgttcttatgggaattgttagcaatgcccttatgggaatttttaacttcacggagcttattcaaatggagagcacttcattttctcgtgatgacatagtgctggatcttggttttatagatgggtccatatttttgttgttgatcacaaactgcgtttctccttttatcggcatgagcagcatcagcgattataaaaaaaatgttcaatcccagttatggatttcaggcctctggccttcagcatactggtgtggacaggctctggtggacattccattatacttcttgattctcttttcaatacatttaatttactacttcatatttctgggattccagctttcatgggaactcatgtttgttttggtggtatgcataattggttgtgcagtttctcttatattcctcacatatgtgctttcattcatctttcgcaagtggagaaaaaataatggcttttggtcttttggcttttttattatcttaatatgtgtatccacaattatggtatcaactcaatatgaaaaactcaacttaattttgtgcatgattttcataccttccttcactttgctggggtatgtcatgttattgatccagctcgactttatgagaaacttggacagtctggacaatagaataaatgaagtcaataaaaccattcttttaacaaccttaataccataccttcagagtgttattttcctttttgtcataaggtgtctggaaatgaagtatggaaatgaaataatgaataaagacccagttttcagaatctctccacggagtagagaaactcatcccaatccggaagagcccgaagaagaagatgaagatgttcaagctgaaagagtccaagcagcaaatgcactcactgctccaaacttggaggaggaaccagtcataactgcaagctgtttacacaaggaatattatgagacaaagaaaagttgcttttcaacaagaaagaagaaaatagccatcagaaatgtttccttttgtgttaaaaaaggtgaagttttgggattactaggacacaatggagctggtaaaagtacttccattaaaatgataactgggtgcacaaagccaactgcaggagtggtggtgttacaaggcagcagagcatcagtaaggcaacagcatgacaacagcctcaagttcttggggtactgccctcaggagaactcactgtggcccaagcttacaatgaaagagcacttggagttgtatgcagctgtgaaaggactgggcaaagaagatgctgctctcagtatttcacgattggtggaagctcttaagctccaggaacaacttaaggctcctgtgaaaactctatcagagggaataaagagaaagctgtgctttgtgctgagcatcctggggaacccatcagtggtgcttctagatgagccgttcaccgggatggaccccgaggggcagcagcaaatgtggcagatacttcaggctaccgttaaaaacaaggagaggggcaccctcttgaccacccattacatgtcagaggctgaggctgtgtgtgaccgtatggccatgatggtgtcaggaacgctaaggtgtattggttccattcaacatctgaaaaacaagtttggtagagattatttactagaaataaaaatgaaagaacctacccaggtggaagctctccacacagagattttgaagcttttcccacaggctgcttggcaggaaagatattcctctttaatggcgtataagttacctgtggaggatgtccaccctctatctcgggcctttttcaagttagaggcgatgaaacagaccttcaacctggaggaatacagcctctctcaggctaccttggagcaggtattcttagaactctgtaaagagcaggagctgggaaatgttgatgataaaattgatacaacagttgaatggaaacttctcccacaggaagacccttaaaatgaagaacctcctaacattcaattttaggtcctactacattgttagtttccataattctacaagaatgtttccttttacttcagttaacaaaagaaaacatttaataaacattcaataatgattacagttttcatttttaaaaatttaggatgaaggaaacaaggaaatatagggaaaagtagtagacaaaattaacaaaatcagacatgttattcatccccaacatgggtctattttgtgcttaaaaataatttaaaaatcatacaatattaggttggttatcggttattatcaataaagctaacactgagaacattttacaaataaaaatatgaggtttttagcctgaacttcaaatgtatcagctatttttaaacattatttactcggattctaatttaatgtgacattgactataagaaggtctgataaactgatgaaatggcacagcataacatttaattataatgacattctgattataaaataaatgcatgtgaattttagtacatattgaagttatatggaagaagatagccataatctgtaagaaagtaccgcagttaatattttctttagccaacttatattcaatgtattttttatggatcctttttcaaaggtagtatcagtaggcatagtcattttctgtatcttttcacctcacagttcatgaacatttcccatgtcattatagcacttttgtgttatataattgctgcattaatgttatagctgtattgatgtaataccagagttgttacgttcgggttatatgcaagtttatttcttagaaataaaactttgatggacttttaaaaaaaaaaaaaaaaa

SEQ ID NO: 49 - RNA, 1892 nt, Homo sapiens
  source 1..1892: mol_type = mRNA
aaaccggtgccaacgtgcgcggacgccgccgccgccgccgccgctggagtccgccgggcagagccggccgcggagcccggagcaggcggagggaagtgcccctagaaccagctcagccagcggcgcttgcacagagcggccggacgaagagcagcgagaggaggaggggagagcggctcgtccacgcgccctgcgccgccgccggcccgggaaggcagcgaggagccggcgcctcccgcgccccgcggtcgccctggagtaatttcggatgcccagccgcggccgccttccccagtagacccgggagaggagttgcggccaacttgtgtgcctttcttccgccccggtgggagccggcgctgcgcgaagggctctcccggcggctcatgctgccggccctgcgcctgcccagcctcgggtgagccgcctccggagagacgggggagcgcggcggcgccgcgggctcggcgtgctctcctccggggacgcgggacgaagcagcagccccgggcgcgcgccagaggcatggagcgctgccccagcctaggggtcaccctctacgccctggtggtggtcctggggctgcgggcgacaccggccggcggccagcactatctccacatccgcccggcacccagcgacaacctgcccctggtggacctcatcgaacacccagaccctatctttgaccccaaggaaaaggatctgaacgagacgctgctgcgctcgctgctcgggggccactacgacccaggcttcatggccacctcgccccccgaggaccggcccggcgggggcgggggtgcagctgggggcgcggaggacctggcggagctggaccagctgctgcggcagcggccgtcgggggccatgccgagcgagatcaaagggctagagttctccgagggcttggcccagggcaagaagcagcgcctaagcaagaagctgcggaggaagttacagatgtggctgtggtcgcagacattctgccccgtgctgtacgcgtggaacgacctgggcagccgcttttggccgcgctacgtgaaggtgggcagctgcttcagtaagcgctcgtgctccgtgcccgagggcatggtgtgcaagccgtccaagtccgtgcacctcacggtgctgcggtggcgctgtcagcggcgcgggggccagcgctgcggctggattcccatccagtaccccatcatttccgagtgcaagtgctcgtgctagaactcgggggccccctgcccgcacccggacacttgatcgatccccaccgacgccccctgcaccgcctccaaccagttccaccaccctctagcgagggttttcaatgaacttttttttttttttttttttttttttctgggctacagagacctagctttctggttcctgtaatgcactgtttaactgtgtaggaatgtatatgtgtgtgtatatacggtcccagttttaatttacttattaaaaggtcagtattatacgttaaaagttaccggcttctactgtatttttaaaaaaaagtaagcaaaagaaaaaaaaaagaacagagaaaagagagacttattctggttgttgctaataatgttaacctgctatttatattccagtgcccttcgcatggcgaagcaggggggaaaagttatttttttcttgaagtacaaagagacgggggaacttttgtagaggactttttaaaagctattttccattcttcggaaagtgttttggttttccttggacctcgaagaagctatagagttcaatgttattttacagttattgtaaatatagagaacaaatggaatgactaatcattgtaaattaagagtatctgctatttattctttataatatcccgtgtagtaaatgagaaagaagtgcagagcaggatt

SEQ ID NO: 50 - RNA, 3227 nt, Homo sapiens
  source 1..3227: mol_type = mRNA
cccactctgcagttgtctcccgagcgctggctgcgccgcccgagccgctgggccggggaagcactggccgttcgctcccgggccggctccgccaggcgctcgcaggcatgcagcccgggagcaggaggcgctccccgggccgctgctgagccggccggggcggcggggaccagcgccagcggagcccctcccaccttgccccggggcagacgagcggcgccccgacaccccctcttctcccgcagccccgccagcgccaccccccgcgggccgcaggggctcatgcagccgccaagggagaggctagtggtaacaggccgagctggatggatgggtatggggagaggggcaggacgttcagccctgggattctggccgaccctcgccttccttctctgcagcttccccgcagccacctccccgtgcaagatcctcaagtgcaactctgagttctggagcgccacgtcgggcagccacgccccagcctcagacgacacccccgagttctgtgcagccttgcgcagctacgccctgtgcacgcggcggacggcccgcacctgccggggtgacctggcctaccactcggccgtccatggcatagaggacctcatgagccagcacaactgctccaaggatggccccacctcgcagccacgcctgcgcacgctcccaccggccggagacagccaggagcgctcggacagccccgagatctgccattacgagaagagctttcacaagcactcggccacccccaactacacgcactgtggcctcttcggggacccacacctcaggactttcaccgaccgcttccagacctgcaaggtgcagggcgcctggccgctcatcgacaataattacctgaacgtgcaggtcaccaacacgcctgtgctgcccggctcagcggccactgccaccagcaagctcaccatcatcttcaagaacttccaggagtgtgtggaccagaaggtgtaccaggctgagatggacgagctcccggccgccttcgtggatggctctaagaacggtggggacaagcacggggccaacagcctgaagatcactgagaaggtgtcaggccagcacgtggagatccaggccaagtacatcggcaccaccatcgtggtgcgccaggtgggccgctacctgacctttgccgtccgcatgccagaggaagtggtcaatgctgtggaggactgggacagccagggtctctacctctgcctgcggggctgccccctcaaccagcagatcgacttccaggccttccacaccaatgctgagggcaccggtgcccgcaggctggcagccgccagccctgcacccacagcccccgagaccttcccatacgagacagccgtggccaagtgcaaggagaagctgccggtggaggacctgtactaccaggcctgcgtcttcgacctcctcaccacgggcgacgtgaacttcacactggccgcctactacgcgttggaggatgtcaagatgctccactccaacaaagacaaactgcacctgtatgagaggactcgggacctgccaggcagggcggctgcggggctgcccctggccccccggcccctcctgggcgccctcgtcccgctcctggccctgctccctgtgttctgctagacgcgtagatgtggagggaggcgcgggctccgtcctctcggcttccccatgtgtgggctgggaccgcccacggggtgcagatctcctggcgtgtccaccatggccccgcagaacgccagggaccgcctgctgccaagggctcaggcacggacccctccccttctagtgcacgtgacaaggttgtggtgactggtgccatgatgtttgacagtagagctgtgtgagagggagagcagctcccctcgccccgcccctgcagtgtgaatgtgtgaaacatcccctcaggctgaagccccccacccccaccagagacacactgggaaccgtcagagtcagctccttccccctcgcaatgcactgaaaggcccggccgactgctgctcgccgatccgtggggccccctgtgcccgccacacgcacgcacacactcttacacgagagcacactcgatccccctaggccagcggggacaccccagccacacagggaggcatccttggggcttggccccaggcagggcaaccccggggcgctgcttggcaccttagcagactgctggaaccttttggccagtaggtcgtgcccgcctggtgccttctggcctgtggcctccctgcccatgttcacctggctgctgtgggtaccagtgcaggtcccggttttcaggcacctgctcagctgcccgtctctggcctgggcccctgccccttccaccctgtgcttagaaagtcgaagtgcttggttctaaatgtctaaacagagaagagatccttgacttctgttcctctctctcctgcagatgcaagagctcctgggcaggggtgcctgggccccagggtgtggcaggagacccagtggatggggccagctggcctgccctgatcctctgcttcctcctcacaaccccaagagcccccagcccggtccatccacgtctggagtctggggagaggagcagggtcttaggactctcagctctgagcatccctggcagggtcttcaacctctaatctcttcccttaagccctgtggccacacagccaggagagacttgccgctggctcccgcctcatttcagcccagggtgctcatccaggggcccagaacagtcccacctgtgctgctgtgcccacagcacaaagccaggcttcactcccaaaagtgcagccaggccctggagggtgatcctgccagcagccctacagctccacaccctacccacccatcggcagcccctctgctgttccccagggacctctcatacactggccaggaggctgcagaacgtgtgtctccccctccctccaagaggtcctgctccctctgccagaaccgtgtgtgggcgggtgggagggcgctcggggcccggcccctccctctccctgctggttttagttggtccctatgttggaagtaaaaagtgaagcactttattttggttgtgtttgctcacgttctgcttggaagtggggacccctcactgcgtccacgtgtctgcgacctgtgtggagtgtcaccgcgtgtacatactgtaaattatttattaatggctaaatgcaagtaaagtttggtttttttgttattttctttta

SEQ ID NO: 51 - RNA, 3200 nt, Homo sapiens
  source 1..3200: mol_type = mRNA
ccatactgaagccctcccaagtgcagccttgcgggcctcgcagagagcgccaaaccatccggccctgcgcgccacgcggaccggcatagccatctctctggagtggcagctgtgccaaggtggcaaggttaggcccgcaggccctcagcacgggggcgcagccggggcaagtcttcaggaagcagcgaggtgcttgaagggggtgctggaggcaggccaaacccagtcaggatgggtggcctggggccacgacgggcgggaacctcgagggagaggctagtggtaacaggccgagctggatggatgggtatggggagaggggcaggacgttcagccctgggattctggccgaccctcgccttccttctctgcagcttccccgcagccacctccccgtgcaagatcctcaagtgcaactctgagttctggagcgccacgtcgggcagccacgccccagcctcagacgacacccccgagttctgtgcagccttgcgcagctacgccctgtgcacgcggcggacggcccgcacctgccggggtgacctggcctaccactcggccgtccatggcatagaggacctcatgagccagcacaactgctccaaggatggccccacctcgcagccacgcctgcgcacgctcccaccggccggagacagccaggagcgctcggacagccccgagatctgccattacgagaagagctttcacaagcactcggccacccccaactacacgcactgtggcctcttcggggacccacacctcaggactttcaccgaccgcttccagacctgcaaggtgcagggcgcctggccgctcatcgacaataattacctgaacgtgcaggtcaccaacacgcctgtgctgcccggctcagcggccactgccaccagcaagctcaccatcatcttcaagaacttccaggagtgtgtggaccagaaggtgtaccaggctgagatggacgagctcccggccgccttcgtggatggctctaagaacggtggggacaagcacggggccaacagcctgaagatcactgagaaggtgtcaggccagcacgtggagatccaggccaagtacatcggcaccaccatcgtggtgcgccaggtgggccgctacctgacctttgccgtccgcatgccagaggaagtggtcaatgctgtggaggactgggacagccagggtctctacctctgcctgcggggctgccccctcaaccagcagatcgacttccaggccttccacaccaatgctgagggcaccggtgcccgcaggctggcagccgccagccctgcacccacagcccccgagaccttcccatacgagacagccgtggccaagtgcaaggagaagctgccggtggaggacctgtactaccaggcctgcgtcttcgacctcctcaccacgggcgacgtgaacttcacactggccgcctactacgcgttggaggatgtcaagatgctccactccaacaaagacaaactgcacctgtatgagaggactcgggacctgccaggcagggcggctgcggggctgcccctggccccccggcccctcctgggcgccctcgtcccgctcctggccctgctccctgtgttctgctagacgcgtagatgtggagggaggcgcgggctccgtcctctcggcttccccatgtgtgggctgggaccgcccacggggtgcagatctcctggcgtgtccaccatggccccgcagaacgccagggaccgcctgctgccaagggctcaggcacggacccctccccttctagtgcacgtgacaaggttgtggtgactggtgccatgatgtttgacagtagagctgtgtgagagggagagcagctcccctcgccccgcccctgcagtgtgaatgtgtgaaacatcccctcaggctgaagccccccacccccaccagagacacactgggaaccgtcagagtcagctccttccccctcgcaatgcactgaaaggcccggccgactgctgctcgccgatccgtggggccccctgtgcccgccacacgcacgcacacactcttacacgagagcacactcgatccccctaggccagcggggacaccccagccacacagggaggcatccttggggcttggccccaggcagggcaaccccggggcgctgcttggcaccttagcagactgctggaaccttttggccagtaggtcgtgcccgcctggtgccttctggcctgtggcctccctgcccatgttcacctggctgctgtgggtaccagtgcaggtcccggttttcaggcacctgctcagctgcccgtctctggcctgggcccctgccccttccaccctgtgcttagaaagtcgaagtgcttggttctaaatgtctaaacagagaagagatccttgacttctgttcctctctctcctgcagatgcaagagctcctgggcaggggtgcctgggccccagggtgtggcaggagacccagtggatggggccagctggcctgccctgatcctctgcttcctcctcacaaccccaagagcccccagcccggtccatccacgtctggagtctggggagaggagcagggtcttaggactctcagctctgagcatccctggcagggtcttcaacctctaatctcttcccttaagccctgtggccacacagccaggagagacttgccgctggctcccgcctcatttcagcccagggtgctcatccaggggcccagaacagtcccacctgtgctgctgtgcccacagcacaaagccaggcttcactcccaaaagtgcagccaggccctggagggtgatcctgccagcagccctacagctccacaccctacccacccatcggcagcccctctgctgttccccagggacctctcatacactggccaggaggctgcagaacgtgtgtctccccctccctccaagaggtcctgctccctctgccagaaccgtgtgtgggcgggtgggagggcgctcggggcccggcccctccctctccctgctggttttagttggtccctatgttggaagtaaaaagtgaagcactttattttggttgtgtttgctcacgttctgcttggaagtggggacccctcactgcgtccacgtgtctgcgacctgtgtggagtgtcaccgcgtgtacatactgtaaattatttattaatggctaaatgcaagtaaagtttggtttttttgttattttctttta

SEQ ID NO: 52 - RNA, 590 nt, Homo sapiens
  source 1..590: mol_type = mRNA
atcccactgggaagcttcaacatagctgtggaagtctgcagtctacaggagcctactatagacattctacaaccaaccagaatcatggaacagccaacttccagcaccaatggggagaagacgaagagcccctgtgaatccaataacaaaaaaaatgatgagatgcaagaggtaccaaacagagtcttagcccccgaacagagtttgaagaacacaaaaacatcagaatatccaataatatttgtgtattacctcaggaagggtaagaaaataaattcaaatcaactggagaatgaacagtcccaagagaactccatcaatccaatccaaaaggaggaggacgaaggcgtagacttatctgaaggatcttcaaatgaggatgaagacctaggcccatgtgaaggaccttcaaaggaggacaaagatctagactcatctgaaggatcctcacaggaggatgaagacctaggcttatctgaaggatcttcacaggacagtggggaggattagtcacacatggagaaaccaaattggacaaatcatcaccactgatggcgatgattacaataaaatcaagtttaaggagctga

SEQ ID NO: 53 - RNA, 1408 nt, Homo sapiens
  source 1..1408: mol_type = mRNA
caccttcctcccatcttgccttctccctcgagttgggacccgggaagaaccatgaagtggctgctgctgctgggtctggtggcgctctctgagtgcatcatgtacaaggtccccctcatcagaaagaagtccttgaggcgcaccctgtccgagcgtggcctgctgaaggacttcctgaagaagcacaacctcaacccagccagaaagtacttcccccagtgggaggctcccaccctggtagatgaacagcccctggagaactacctggatatggagtacttcggcactatcggcatcggaactcctgcccaggatttcaccgtcgtctttgacaccggctcctccaacctgtgggtgccctcagtctactgctccagtcttgcctgcaccaaccacaaccgcttcaaccctgaggattcttccacctaccagtccaccagcgagacagtctccatcacctacggcaccggcagcatgacaggcatcctcggatacgacactgtccaggttggaggcatctctgacaccaatcagatcttcggcctgagcgagacggaacctggctccttcctgtattatgctcccttcgatggcatcctggggctggcctaccccagcatttcctcctccggggccacacccgtctttgacaacatctggaaccagggcctggtttctcaggacctcttctctgtctacctcagcgccgatgacaagagtggcagcgtggtgatctttggtggcattgactcttcttactacactggaagtctgaactgggtgcctgttaccgtcgagggttactggcagatcaccgtggacagcatcaccatgaacggagagaccatcgcctgtgctgagggctgccaggccattgttgacaccggcacctctctgctgaccggcccaaccagccccattgccaacatccagagcgacatcggagccagcgagaactcagatggcgacatggtggtcagctgctcagccatcagcagcctgcccgacatcgtcttcaccatcaatggagtccagtaccccgtgccacccagtgcctacatcctgcagagcgaggggagctgcatcagtggcttccagggcatgaacgtccccaccgaatctggagagctttggatcctgggtgatgtcttcatccgccagtactttaccgtcttcgacagggcaaacaaccaggtcggcctggcccctgtggcttaagcctaagtctcttcagccacctcccaggaagatctggcctccgtcctatgcccactttagatgtatctaattctcctgactgttcttcccaggggagtgtgaaggtcttggccctgttccctgtcctaccaataacgtagaataaaaacataacccactgaaaaaaaaaaaaaaaaaaaaaaaaaaaaaa

SEQ ID NO: 54 - RNA, 5073 nt, Homo sapiens
  source 1..5073: mol_type = mRNA
aggctggccctggctgcctgcggcgcgggcgcctccctcgcagccgctgctgccgacgccgctgcgctcccgcctcctgtcggttcccgggttcccgctgcggctgcggttctggcagccgagcccccgcggtgctgcagcccagctttagcgcgcagaccgacccgcgccccttcttcgccgccggcagcctctaatccacgcggcgcgttgcggcaggtgccctgggcgtactgaggcgcggtggcctgagcccggccgccatcgatgaccccggtcgcggacttgcttcaggctggccaccccccgtcttgtttcatcatctgtgttgagtaaccatggggaggaagctggacctgtctggtttgactgatgatgaaacagagcatgttcttcaggtggttcaaagagacttcaatcttcgcaaaaaagaagaagaacgactaagtgagctgaagcagaagctggatgaggaaggcagcaagtgcagcatcctctcgaagcaccagcagtttgtggagcactgctgcatgcgctgctgctcgcccttcaccttcctcgtcaacaccaagcgccagtgtggagattgcaaattcaatgtctgcaagagctgctgctcctaccagaagcacgaaaaggcctgggtctgctgcgtctgccagcaagcgaggcttctgagggcccaatctctggaatggttctacaataatgtgaagagccgcttcaagcgctttggcagtgccaaggttctgaagaacctgtacaggaagcaccggctggagagtggcgcgtgcttcgacattctaggaggaagcctttttgagtcaaacctggagaatgaaggaagcatttctggcagtgattcaacattttataggcagtcagaaggacatagtgtgatggacaccttggctgtggccctacgggtggctgaagaggccattgaggaagcaatttccaaagcagaggcatatggggacagcctggacaagcaaaatgaggccagttacctgcgggaccacaaggaggagctaactgaggaactggccacgacaatcctgcagaagattatacgaaaacagaagagcaaaagtgagcagcaagtggaagaagagccaggatggccacatccccagagttgcagcacaaaggtggcagatgaggggacctcagcatcccctggaggctaccgtgctcccgctgccctctggaggtcccagtctgccttctcaatcactggagaagaagccctgaagacccctccagtggaggctccatcgaggcagccaagggaccaaggccaacacccgagagcagagtctgctctgcccagctggaagagtgtggacaggctggatgaaacaaacctggccccagttttgcagagccccgacgggaactgggtggccctgaaggatggcgctccaccccccacccgactactggccaaacctaagagcgggacgtttcaggccctggaggtggcctccagtgtggcatctgcctacgatgagatgggctccgatagcgaggaagactttgactggagtgaggccttgagcaagctgtgtcccaggtcccgggccctgcccaggaacccccagcctcagcccacacaggcccagagctctgaccaaggccccatagctgcctccccatcctctgcactctcccccaaccctgaggccatgtgctctgactcggagacctcctccgcaggctcttcccgagaagttgggcaccaggccagactgtcctggttgcagaggaaggcccccaggaaccctgcagctgagaagatgcgcttgcatggagagctggacgtgaacttcaacccccagttggccagcagggagacctcggacagcagcgagccggaggaggccccccacaccacagaccggcgggccaggaggtggagaagagcccgactgggctcagaagagccaagcaaagaaccatcttcccccagcgcccagctccgggatctagacacacatcaggtgtcggatgatttatcagagacagacatcagcaatgaggctcgggatccccagactctcacagacaccacagaggagaaacggagaaacaggctgtacgagttagcaatgaaaatgagtgaaaaggagacttcttcaggggaggatcaggagtctgagcccaagacagaatctgagaaccagaaggaaagtctgtcctctgaagacaacagccagagtgtccaggaagagctgaagaagaagttttctgctgtttctctctgcaacatctccacagaagtcctgaaagtcatcaatgccacagaggagttgatagcaggatctacagggccctgggagtccccacaagtccctcctgacagacagaaggggatgtttcctcgtgggacagaccaagtgagactggatgagcagctgacttccctggaagaaaatgtatacctggcagcaggcactgtgtatggactggagacccagctgactgagctagaagatgccgcccgctgcatccacagtggcactgatgagacccatctggcggatctggaggaccaggtggccacggctgcagcccaagtccaccatgctgaactccagatttcagatattgagagccggatttcagccctgaccattgcaggattaaacatagcaccatgtgtgcgcttcacaagaagacgggatcagaagcaaaggacccaggtacaaaccatagatacatcaaggcagcaaaggaggaaactgcctgctccaccggtgaaagctgaaaaaattgagacatcttcagtgactaccattaaaacatttaaccacaacttcattctccaaggctcctcaacaaacaggactaaggaaaggaaaggcaccaccaaggatttgatggagcctgctctggagtcagctgtgatgtactgacaccatggaattccactgccagtgacccactgcctccggccgtacacgacagtgccttgacccaacagccatcgagtactgtatgtatttccacctgaggagaaggcctggggaggccacagtgcaccattgcacagggctgtcctgatacctcatccagaaagccgtctcagacttcagcactgcggtcttgcccactctctgccttaggctcccaggggaatccaagacagaaaatgaagacactggcttccaacagcagcgctccatgtttaagatacatattttccctgtttgctttgctactgtatgttgactttaagatctttttttaaatacatttgattcagctagtattccatgtcaacaatttgtccaaaggaaaactgctggagggaggtggagggaggaaggtgggaattattatttaatacatcattaatgcttattaatctctcacaagcatctttgtcttgcaaatcctaagggaaaagcaagtccctgcagtgagcactagggacagtctaatttggggattgctcaaccatcaagactgcaggtctcccttcagccacctccttcctgctaaaagcttagcctaccacactaccagtcattcccatcgctttgcaatcacaagccacaggatgagaagttctgactcactcatgccatgcccagggctatctgaaacaatgtctcattaagaatttagggttcttccatgggcttactgacagttgcccagatctgaaggggaaagggtcttgagaaagaccatcactggctcaactttagggcactgtccagagtcaacatgatgtggtttagcagtgatcacatctaaacaaagtttaggtaaatgaattatcgcagagaaaaaccacatgagaaaatttttgtactccaaatttacttcccaataaatattcagcaaagtagtaaaatgaccttaaagataaaaatgattagggaatagccttagaaaatttataggtataaaaaattcaaggacaaactgtgcatttaatggacacaagaattgactctaactccatgtctgtggtttctttgaacccatatcaaatgtatgactatttagagtgtttataagagataatggaactgaactttcactcaattaattgggcattaacaaccttcttttatgtttgttcctgatatagtctgaatcttaggaagaaggtaaaagaaaggaggcaagagaatagttatgatgaatatgtgttaagtgcctgctctgaaggaggcaatgttcttctcatttgaatccttatggcaaccttattcaataggttttcccatatttcagatttaataactgaaggccagagagattaatttgccaaagccacacctttatgctaattatgattggaatgcatcacaaaagcctaactctgttgttttcaacctctacgttattttgctgctatgtgcatttccagatctgattttctgctaacttgtgtgctatgatccactcctgatgggggtctacattaatcttccagtactccttgctgatgctgtgttatgtgtcatctaacagaaatgactcctttgaaataagtaaatctttggctttttgttctgttggtgtgattcaaagcaaaacaaacaaacaaaaacaaattttaagaacacaacaaaaaagatttgacttccgaatagaatgttttctttaagaggcatgaaaagcaactattgttgtgttacagtgttaaaaatattcagttttctttgacaaaaatgtgtactgtgtaagccttgcaaacaaaaaacaacaaaaaagaagcagcagcagcagcctgctgtgtggcatctgaacttttataaaggtttccttgtgccaaataagtgcaaagatttaatttactattaaaaaccataagcatatgttatagttccagaagaattattttgtcatcaagtgattttgatctttagtgtcaatatttatatttagattaatttttataaatgaaaatattttaatggtttaagaaaatgaggacaacaggataatatctttgatgacttctgaaagttatgcttcccttcatgttatatgcacattgccaagaattactgtcaagagaaatgataagtaaaagtcatttatgaaaataaa

SEQ ID NO: 55 - RNA, 4857 nt, Homo sapiens
  source 1..4857: mol_type = mRNA
aacccggcggttccgcagctgtgtttgggagacttgggggcgcattagcctggacagctccctgatcggtcttgtttcatcatctgtgttgagtaaccatggggaggaagctggacctgtctggtttgactgatgatgaaacagagcatgttcttcaggtggttcaaagagacttcaatcttcgcaaaaaagaagaagaacgactaagtgagctgaagcagaagctggatgaggaaggcagcaagtgcagcatcctctcgaagcaccagcagtttgtggagcactgctgcatgcgctgctgctcgcccttcaccttcctcgtcaacaccaagcgccagtgtggagattgcaaattcaatgtctgcaagagctgctgctcctaccagaagcacgaaaaggcctgggtctgctgcgtctgccagcaagcgaggcttctgagggcccaatctctggaatggttctacaataatgtgaagagccgcttcaagcgctttggcagtgccaaggttctgaagaacctgtacaggaagcaccggctggagagtggcgcgtgcttcgacattctaggaggaagcctttttgagtcaaacctggagaatgaaggaagcatttctggcagtgattcaacattttataggcagtcagaaggacatagtgtgatggacaccttggctgtggccctacgggtggctgaagaggccattgaggaagcaatttccaaagcagaggcatatggggacagcctggacaagcaaaatgaggccagttacctgcgggaccacaaggaggagctaactgaggaactggccacgacaatcctgcagaagattatacgaaaacagaagagcaaaagtgagcagcaagtggaagaagagccaggatggccacatccccagagttgcagcacaaaggtggcagatgaggggacctcagcatcccctggaggctaccgtgctcccgctgccctctggaggtcccagtctgccttctcaatcactggagaagaagccctgaagacccctccagtggaggctccatcgaggcagccaagggaccaaggccaacacccgagagcagagtctgctctgcccagctggaagagtgtggacaggctggatgaaacaaacctggccccagttttgcagagccccgacgggaactgggtggccctgaaggatggcgctccaccccccacccgactactggccaaacctaagagcgggacgtttcaggccctggaggtggcctccagtgtggcatctgcctacgatgagatgggctccgatagcgaggaagactttgactggagtgaggccttgagcaagctgtgtcccaggtcccgggccctgcccaggaacccccagcctcagcccacacaggcccagagctctgaccaaggccccatagctgcctccccatcctctgcactctcccccaaccctgaggccatgtgctctgactcggagacctcctccgcaggctcttcccgagaagttgggcaccaggccagactgtcctggttgcagaggaaggcccccaggaaccctgcagctgagaagatgcgcttgcatggagagctggacgtgaacttcaacccccagttggccagcagggagacctcggacagcagcgagccggaggaggccccccacaccacagaccggcgggccaggaggtggagaagagcccgactgggctcagaagagccaagcaaagaaccatcttcccccagcgcccagctccgggatctagacacacatcaggtgtcggatgatttatcagagacagacatcagcaatgaggctcgggatccccagactctcacagacaccacagaggagaaacggagaaacaggctgtacgagttagcaatgaaaatgagtgaaaaggagacttcttcaggggaggatcaggagtctgagcccaagacagaatctgagaaccagaaggaaagtctgtcctctgaagacaacagccagagtgtccaggaagagctgaagaagaagttttctgctgtttctctctgcaacatctccacagaagtcctgaaagtcatcaatgccacagaggagttgatagcaggatctacagggccctgggagtccccacaagtccctcctgacagacagaaggggatgtttcctcgtgggacagaccaagtgagactggatgagcagctgacttccctggaagaaaatgtatacctggcagcaggcactgtgtatggactggagacccagctgactgagctagaagatgccgcccgctgcatccacagtggcactgatgagacccatctggcggatctggaggaccaggtggccacggctgcagcccaagtccaccatgctgaactccagatttcagatattgagagccggatttcagccctgaccattgcaggattaaacatagcaccatgtgtgcgcttcacaagaagacgggatcagaagcaaaggacccaggtacaaaccatagatacatcaaggcagcaaaggaggaaactgcctgctccaccggtgaaagctgaaaaaattgagacatcttcagtgactaccattaaaacatttaaccacaacttcattctccaaggctcctcaacaaacaggactaaggaaaggaaaggcaccaccaaggatttgatggagcctgctctggagtcagctgtgatgtactgacaccatggaattccactgccagtgacccactgcctccggccgtacacgacagtgccttgacccaacagccatcgagtactgtatgtatttccacctgaggagaaggcctggggaggccacagtgcaccattgcacagggctgtcctgatacctcatccagaaagccgtctcagacttcagcactgcggtcttgcccactctctgccttaggctcccaggggaatccaagacagaaaatgaagacactggcttccaacagcagcgctccatgtttaagatacatattttccctgtttgctttgctactgtatgttgactttaagatctttttttaaatacatttgattcagctagtattccatgtcaacaatttgtccaaaggaaaactgctggagggaggtggagggaggaaggtgggaattattatttaatacatcattaatgcttattaatctctcacaagcatctttgtcttgcaaatcctaagggaaaagcaagtccctgcagtgagcactagggacagtctaatttggggattgctcaaccatcaagactgcaggtctcccttcagccacctccttcctgctaaaagcttagcctaccacactaccagtcattcccatcgctttgcaatcacaagccacaggatgagaagttctgactcactcatgccatgcccagggctatctgaaacaatgtctcattaagaatttagggttcttccatgggcttactgacagttgcccagatctgaaggggaaagggtcttgagaaagaccatcactggctcaactttagggcactgtccagagtcaacatgatgtggtttagcagtgatcacatctaaacaaagtttaggtaaatgaattatcgcagagaaaaaccacatgagaaaatttttgtactccaaatttacttcccaataaatattcagcaaagtagtaaaatgaccttaaagataaaaatgattagggaatagccttagaaaatttataggtataaaaaattcaaggacaaactgtgcatttaatggacacaagaattgactctaactccatgtctgtggtttctttgaacccatatcaaatgtatgactatttagagtgtttataagagataatggaactgaactttcactcaattaattgggcattaacaaccttcttttatgtttgttcctgatatagtctgaatcttaggaagaaggtaaaagaaaggaggcaagagaatagttatgatgaatatgtgttaagtgcctgctctgaaggaggcaatgttcttctcatttgaatccttatggcaaccttattcaataggttttcccatatttcagatttaataactgaaggccagagagattaatttgccaaagccacacctttatgctaattatgattggaatgcatcacaaaagcctaactctgttgttttcaacctctacgttattttgctgctatgtgcatttccagatctgattttctgctaacttgtgtgctatgatccactcctgatgggggtctacattaatcttccagtactccttgctgatgctgtgttatgtgtcatctaacagaaatgactcctttgaaataagtaaatctttggctttttgttctgttggtgtgattcaaagcaaaacaaacaaacaaaaacaaattttaagaacacaacaaaaaagatttgacttccgaatagaatgttttctttaagaggcatgaaaagcaactattgttgtgttacagtgttaaaaatattcagttttctttgacaaaaatgtgtactgtgtaagccttgcaaacaaaaaacaacaaaaaagaagcagcagcagcagcctgctgtgtggcatctgaacttttataaaggtttccttgtgccaaataagtgcaaagatttaatttactattaaaaaccataagcatatgttatagttccagaagaattattttgtcatcaagtgattttgatctttagtgtcaatatttatatttagattaatttttataaatgaaaatattttaatggtttaagaaaatgaggacaacaggataatatctttgatgacttctgaaagttatgcttcccttcatgttatatgcacattgccaagaattactgtcaagagaaatgataagtaaaagtcatttatgaaaataaaaaaaaaaaaaaaaaaaaaaaaaaa

SEQ ID NO: 56 - RNA, 1473 nt, Homo sapiens
  source 1..1473: mol_type = mRNA
cttcaacactgtggaagctttgttctttcgctcttttgcaataaatcttgctactgctcactctttgggtccacactgcctttatgagctgtaacactcaccgcgaaaggtctgcagcttcactcctgaagccagcgagcccacgagcccacagggaggaatgaacaactccagatgcaccgccttaagagctgtaacactcacggcgaaggtctgcagcttcactcctgagccagcgagaccaggaacccaccagaaggaagaaactccgaacacatccgaacatcagaaggaacaaactccagacggcgccaccttaagagctgtaacactcaccgccagggtccggggcttcgttcttgaagtcagtgagaccaagaacccaccaattccggacgcagtaccatgatcaacaggatgttactagcaacttccttggagcgatgtggttgatatcaataacttttctctccattggttatggtgacatggtacctaacacatactgtggaaaaggagtctgcttacttactggaattatgggtgctggttgcacagccctggtggtagctgtagtggcaaggaagctagaacttaccaaagcagaaaaacacgtgcacaatttcatgatggatactcagctgactaaaagagtaaaaaatgcagctgccaatgtactcagggaaacatggctaatttacaaaaatacaaagctagtgaaaaagatagatcatgcaaaagtaagaaaacatcaacgaaaattcctgcaagctattcatcaattaagaagtgtaaaaatggagcagaggaaactgaatgaccaagcaaacactttggtggacttggcaaagacccagaacatcatgtatgatatgatttctgacttaaacgaaaggagtgaagacttcgagaagaggattgttaccctggaaacaaaactagagactttgattggtagcatccacgccctccctgggctcataagccagaccatcaggcagcagcagagagatttcattgaggctcagatggagagctacgacaagcacgtcacttacaatgctgagcggtcccggtcctcgtccaggaggcggcggtcctcttccacagcaccaccaacttcatcagagagtagctagaagagaataagttaaccacaaaataagactttttgccatcatatggtcaatattttagcttttattgtaaagcccctatggttctaatcagcgttatccgggttctgatgtcagaatcctgggaacctgaacactaagttttaggccaaaatgagtgaaaactctttttttttctttcagatgcacagggaatgcacctattattgctatatagattgttcctcctgtaatttcactaactttttattcatgcacttcaaacaaactttactactacattatatgatatataataaaaaaagttaatttctgcacataaaaaaaaaaaaaaaaa

SEQ ID NO: 57 - RNA, 2112 nt, Homo sapiens
  source 1..2112: mol_type = mRNA
cggcggcagcagcccatgcctccggtgcaacagctgcgcctcctccggtgccccggcggcgggggcgggagataacctgtccctgctgctccgcacctcctcgcccggcggcgccttccggacccgcacctcctcgccgctgtcgggctcgtcctgctgctgctgctgctgctcgtcgcgccggggcagccagctcaatgtgagcgagctgacgccgtccagccatgccagtgcgctccggcagcagtacgcgcagcagtccgcgcagcagtcggcgtccgcctcccagtaccaccagtgccacagcctgcagcccgccgccagccccacgggcagcctcggcagtctgggctccgggcccccgctctcgcaccaccaccaccacccgcacccggcgcaccaccagcaccaccagccccaggcgcgccgcgagagcaaccccttcaccgaaatagccatgagcagctgcaggtacaacgggggcgtcatgcggccgctcagcaacttgagcgcgtcccgccggaacctgcacgagatggactcagaggcgcagcccctgcagccccccgcgtctgtcggaggaggtggcggcgcgtcctccccgtctgcagccgctgccgccgccgccgctgtttcgtcctcagcccccgagatcgtggtgtctaagcccgagcacaacaactccaacaacctggcgctctatggaaccggcggcggaggcagcactggaggaggcggcggcggtggcgggagcgggcacggcagcagcagtggcaccaagtccagcaaaaagaaaaaccagaacatcggctacaagctgggccaccggcgcgccctgttcgaaaagcgcaagcggctcagcgactacgcgctcatcttcggcatgttcggcatcgtggtcatggtcatcgagaccgagctgtcgtggggcgcctacgacaaggcgtcgctgtattccttagctctgaaatgccttatcagtctctccacgatcatcctgctcggtctgatcatcgtgtaccacgccagggaaatacaggtaccatgatcaacaggatgttactagcaacttccttggagcgatgtggttgatatcaataacttttctctccattggttatggtgacatggtacctaacacatactgtggaaaaggagtctgcttacttactggaattatgggtgctggttgcacagccctggtggtagctgtagtggcaaggaagctagaacttaccaaagcagaaaaacacgtgcacaatttcatgatggatactcagctgactaaaagagtaaaaaatgcagctgccaatgtactcagggaaacatggctaatttacaaaaatacaaagctagtgaaaaagatagatcatgcaaaagtaagaaaacatcaacgaaaattcctgcaagctattcatcaattaagaagtgtaaaaatggagcagaggaaactgaatgaccaagcaaacactttggtggacttggcaaagacccagaacatcatgtatgatatgatttctgacttaaacgaaaggagtgaagacttcgagaagaggattgttaccctggaaacaaaactagagactttgattggtagcatccacgccctccctgggctcataagccagaccatcaggcagcagcagagagatttcattgaggctcagatggagagctacgacaagcacgtcacttacaatgctgagcggtcccggtcctcgtccaggaggcggcggtcctcttccacagcaccaccaacttcatcagagagtagctagaagagaataagttaaccacaaaataagactttttgccatcatatggtcaatattttagcttttattgtaaagcccctatggttctaatcagcgttatccgggttctgatgtcagaatcctgggaacctgaacactaagttttaggccaaaatgagtgaaaactctttttttttctttcagatgcacagggaatgcacctattattgctatatagattgttcctcctgtaatttcactaactttttattcatgcacttcaaacaaactttactactacattatatgatatataataaaaaaagttaatttctgcacataaaaaaaaaaaaaaaaa

SEQ ID NO: 58 - DNA, 36151 bp, Homo sapiens
  source 1..36151: mol_type = genomic DNA
caagctgacttctcaagctctggggatgcctcagtgatctctgatgtggaattagtggaggctggccgttgctcacctctacacagcctgctggtcgttagcgagcaggagttctgatgttcctctcatcttggatggtaagaaatttatgaaaatgctaagtcctgaggattaatagaggaaatgaggactaaatatacaaaatagtccagaaggtggcaggtggaacacagcaataatatatgatgttagtcatcagtcattagtgccacagggatcctaggcgatggctgggaaatggcttttgcaggctgagatggtggtagcgcttcaccctctaaggcaagtgcctatgattcaatgggtgaactcactgccaccccagcagggtggggttggggttggcttggtgagaagggagatgtcatcttgcccaaggaggcttatcccttgtgaaagtctggaacaacacacaaaacaccaggaggaactgtttcggagtgctgtcttgaatgcaagcaggcagcctccatttagatctcactgattcttctaggatattacaaagcactttcttaccccaaatccttcagtgccaccctgccactaaatacaaagaagaagctctgcttcccaccgtgcagaggagccacagggattgcatggtccccatgactgcctctttggcccagggaaagggcccaatcagacagcaccccagatcttaagagaagaacttccagtcaaaacaacagggcacccccgtgtgctggaaggtccaactctctccagtcccaagagtgttaagcatctggctaaggctttgctaaatttcccataagagctgcattgttttcttctgtctgttagacctaggaagttttctgggtgtggacgtagggcttttgcaagtttcaaagcttccaggggattagaaaccatcattcccaagcatttacaagaaaatcttttgtccccactgcttgatatcgaaaaacaagggtcactcttcttttcccctaaggagggaaatgggaacaccccgctgaccatctccttctgcctcaggcactttcatggagacagtcgagggctttggggcctgtcctacctggtggtctactcagtagagccatcgggctgaaaaggagacatctgttaaggtaactggtgatcccatgtaaaagctttgactaaaccacaggagctggaaccactttctcagtaaagcatgccaggaagcacaaataaagtcatgtgctgcataaggacgttttggtcaatgagggactgcataaatgatggaggtcccataaaattataatatcatatttttactgtcccttttctatgtttagataaacaaatattaccattgcattacaactgctcacagtatttcagcaggaaagggcccttcgggaggggctccagcttgcctctccaggtctaggtcttatcgttcttccccttgaagttgaccctacaaccttattaaatcttctgcagttaccaaaagtgataatgtgcttggcctttgtttaagctgtgctctctgccttgagctgtcctccttccctctgctcaagtgccccatttttcatgtcccttgggaacaagctcaggtgtcatcactgaattcaggtagatgcccctcttatctgtccccagagcatgctgcacttatccccatcacagcacttctcatgctctgttataatttccttcctattccattagcatatgaggaaccaagggccatgtgtcattcatcctagtacatgttacttagtggagttgcataaatacttatggaatgaataaattgactaagaggtgagctgggctcagcttgtggatgatcctgaaagatagattggcagactcttaccttttttgggagtgtgcaaccggaaactgtttattgtgtttttgaggtgggagataatttattgggactgtcctttggcatgatagctctagaatgagtgctaaggttgaatgggatggaagagagagccagttagtaagccattgcagggtgcaggtgagacagaataaactgaagttaaataggagtaatgcgggaacattcaaaatagggtcagtaagaagtgatcacaaataacgcaagggagacggaggaatcaagggtgatgtggaggtttccagcgtctactgaagtgagtgaatgaggatgcctctttcccactagaggaagataggtatgggggtggccacagctgcccggttgcatggataggaactccttgacttaccttttattagaagatgggtaatgatgactccatcactgtaactgcaatctattctgggtgaagagtgcccatacggtaaatgttttaaaatattctgaatattgcccctggtcccaagggatgaaggcattgtggaggagttttcccttaagcatagttgaaataggagaaaaaaaaaagaaaaggaaaaatcagaagttatgtcttagaagggtgttgatgtggattggtttaccagggttgctgtaacgaagcagcatggcctgggtggcttgaacaacagaggtttattttctcacagttctggaggctagaagtctgagatcaggctgtcagtgggtttgcatcctcctcaggcctctctccgggcatgtaggtggctgtcatctccctgcgtcctcacagggtctttcctgtgtgggtgtctgtgtcctcatctcttcttctaaggacacaagtttgtttttggattgggatccaccctaattacttcacttaactttaatcacctctttaaagacctacctccaaatagggtcacggtgtgagatactgggaagttaggacttcaatatatgcattttggtggcaggaggcgcacaattcagcccgcaacatgaggcatgagcaaaaatataaatttaaacaatgttggcaaaaacagattcaaaagcaaaatgcaacgccaaagcatgaggaaagggaagaagttttggatagtaggcatggatgaggtggtcccgagggagagaagaggctggggcaccacgcggaggggtttggtagaccctgagtggtttctctcattgtagagggtcaggaacaatttgaacacagaacaactgaagagccaggcttgatggctctgttaaggaaaagacacttttaggacgtgcagttggaccttttcaagaagctgttggaggtcagggtctgagttgagaaaggagcttggtcctgtaagtcatcgacactcagttgcttctggatcccatcctcaccccctgcaccgcggggtccttctcagggaacgggccacttcccgatgctccctgggctgccatcagctgccatgaacactctgcttagtggaggctccgtggcctgtgaattagcatcaacctgaaataacaagcaggggcttcctatgagtcagccatagtctgttcagagatgctgcctaaagggtctaaatccaaaggcattaattaatttgttcccagggtccacagcatggggagctcaagcccttccatttccgctcattgataccggctgggtaatattatgtgggttccatttttaatgtagaatgccttatttgacaaacatccagacagcacccccaactttgttttcttgagcagaagagagaaaacaagagatgaaggcattgatgcatcagccctgcagaaaaatggcaaaggttacaatatgttatatttagatccgcaatttgccgaaggaagataattgggaaattaagttgcctggttgggaaatcagccgtccttttgtttttgtccggttgtgtagtctcataaatgttcagggcttcaatacctttaggcacttataattaattttttaaaaattggaagattcagtatataagctgcctgatttaatgaaataagtcaaaaggagaaaaaagaagggagtttcttgcagtaattggttgttacatttttccacattgccattctaattcattcctttgaaaagagttcgtttttcagattctataagtacccatggcaataagtgctatttataataaagagacataatgagtctcagctgcacccagggaggttgcagcaggtcaggagcctctctgtctgctccattgttgctgggagagagggtcttgttccaagggttgggtgggaaacaggaattccccacactgtccctgaaattgtggagtgatgaactagggagggaagtcttaactggaatttttcaatattagattttccagagacttcattcagcccactcttcagtagggaaataaatcctttatgtagaaaaaaaatcaaaccatttccttttgaataaggtaatctctgaatctgaggaaccccgagataagatgatgtattagcctgctcaggctgtcataacaatgtaccgcagactgggtggcttcaacgtcggagatttatttccttgcagttccggaggccgggagttctagaatacatcaaggcatccacagggttggtgtcttctgagtcctctctcccgggcatgcagggggctgtcatctccctgtgtcctcacatggtcttcaccctgtgtatgtgtgccttactctttgcttaaaaggacatcagtcatattgggttagggtagagcctcattttaccttcactaccattttaaataccctatctccaaacacagtcacattctgaggtactggctctgcatataaatttggggggacacatttcagctcataatagatgtgcatcttatttttgaaaataaaattacagaggtctttcctcttattcccttttcctctttcaccattcctgcctttcctgtattagctgagacagtaattcatattgtcagagcacacactgtctctctctctcacacacaaacacacatacctccacacactttatctttcctgcctccaaattattttcttgttattggaagcaaaaatgcatttttccttcataggcaccttcttacccagtcctcaatgggtgctgtgatcaaaggaggccaccacagctctattagctcatgcccaaataaagccaaatctcacaccttccacaagtgacctgtgttgctcccttcctgaggttgtttcacagagaagagacccaaggttaggctggctgttggcctccatcagtgatagtgatggctgggtcacaggttgctgaaggagtcaagggactcattcaatactggatgcttctgttcctctttcctctggggctggactaattaaggaaaaatgtttcctggctgttcaggtttcctccatgctaattcaggcctattcttgcagatgcatacagttatgacttcattatgcttgttggtatggaaatagaggtaagatcaggtgcccagtggtctgaaaaatgttgacatgcatttttgagcctgtccacagttgtcgttaaagccttgtcagacttccctgggaggacatttagagtgagaaaaaagagaacctaggaaaaattcctgggaaacatcagcatttccagttcagctgcatgcttgcagatgcgaaaaagtcagggaagtggaagccaggaaggtgagaggaaaaccgggatgggaggagctgtggagatcaagggtggggcaagagtttcatcggggaggggcagcagtctgcagtggccagggttgtggatacatgaagcatatgattcctgactaagtgaggatttctggagtgcgtcatctaattttctctgaactcattttgcaagaatttcctagggattccattggggcgggcgaggttccccttgatgctttcatgtagtagttggctcagagggaatggtggaggtaggaggcatatagctcctcttcaagtgccacttcaaatccactaggtgttatctctcattttggctactgagctacatgttgtgcccccgttccagcaccttccagcaggtgtaactgacaatactcaccccaggctcacacacatagcctttgctttgtgctgctgtcttctccattggtatggcatggagcatggccattagcacctgctcagtgctcatgagtgcaccagagttatttccctgtgggcagcttgtgaccagagtaggtcagaagctaatggagaaatgcttcctcctttcctcctctgggaaaaaggtctgcagaattgagcaactggttgcctgtggtgatggccaaatttctgaacacatcattagaatgttagggtgactctctcctcctctgctttgctttctctcacccttggtccatggaccaccctccctactgaagtacttgcaactcaactttgggggaaactgtggataagagaattagtctgggaagagttggattacttaaaagtcaaagaggaatacggaccccattgctggtgataagaggagtggtgataatccttggtatgcaacagcttcctgttactatggctcttgcctgtggtagagtgatgtgtggcacaggtggaaggtaatgcattaacttaggtcagcagctggcaagccatcgtccgtcgcctatttttgtatggcctgtgagtataaaatggcttttgcatttttagaggattggaaccacacacacacacacacacatacacacacacacacacacacacacagaatatgcaacagagactgtgtgtagcctacaaagcctaaaatattttctgtcttccatttactgacgaagtttgctgaactctggtgtaagtgatagggtaccatgtgaacaatgagaacatgaagaatggccatggcagctgacagctaacggctagatagtactagtgaacatgagtaacactcacagaatataagcaataattagacaaggccactgtgtcaccaccatggaacaagacagacaagaccacttcatgactgtgagtgaaacaagatagagacaaggacaccctgcaactccccctccaaataacttaacatgccactcttctaacaagaataagagactatcacttcgtgctgattgcaactctatctgtgattcaatcctcctgcctcctaattaaaaattaccaaggaaccaaatcactgaattgttcacataccctaacagcattcagtctagaactgtctttgtttccttcaactctccctccaatcacctggcacaaggtcaaattctacaaaaatcctatcttaattcctagtttccaagacatcccacagccctacagaaataaagaccacccaactgagaacaaggatggtgatttattcggagcttgctgtagtgaaagagtcggccaccatcactggtgtttggcagagactcaaaggcaggcagaggggtgggagagctttacagtgggcaaaaaagacgtcttcaggtgtgccccaattggaggctgttggcctagagaagctggaggtggccaagtaggagcagggcaggctatgtgattggttggggacatatttgaccttctctggtttgtcctgaattggaagtggggacaaaaatcaagaaatatgtcagctattaatcatgtgctggtcattttgggctgattgctacagaagttgtggctcagagtcttattgccacctctggtccagccactggccatgggtgtgttcagttttcagttctctggaatgccttcttttctctgcagtaagctcaatgaacttggaagcagattctcccccacagcctctagggaagagcccagctatgtcaatgctgatttgggcctgtgagaccctaagctgagaacacagttaaggccccccagacttctgatctccagagttagaaataaatgagcactctttcaagctgctgagtttatgctaatttgtttgacaacaggtgattcctgagggtcactggttactggacttggaaaactgtgtgagtgcaagcataattattaggatcacagtgtatgctgggttttgttaactgcattgacagccttaaagaaaatggtaccctcagatcagccaactgtcaactcaaggtgtgctgtgaaagctggaggcctgtagaaagagtttaaagaaccatgacctcctttagccagaggaagactagatatctacaaagacctcacttgaggctgatccttcctcacaagatggtgttcatcctcctgagggtctttgctgtgaccccttaccatctccagaccaatgaccaggatcaggcctcatagccctgcctgccctgaaaacatagggataaaacagatcccagtggttatttagcaaatgttctgcatcctctatgtctgcatcagttactacctcaaaacagctggcattttgccttttttcccccactaatttaaagcgcattctgagagcaggggtcagcacactctttctttaagggtcagattgtaaatattttcatttctgcaaaccatttggtctttgttgttatcctccactttgccactagtagacatagataatacacaagcgaatgggcatggcttttgttccaatataacttggtttacaaaaacagaaacaggccagatttggcccacaggctatagtgttccagcttcagtcttggaaaatcatttaatctctctgggtttcatttctacacctgtaaaattagagtattgttctaagacaatgcctctcacactccagctagcgttagaatcatgtggagagctactgaaagcacagattcttgcaccttactcccagtgattccagttgaataggtctggagtgggatctgcatttttaacatgctcccaggtaaaactagtgccgctggtccagggaccatgctttgagtagcagaagtcttgggcagtacttctcatccctggcttcagaggagactcgtgctgagaacttttaaaaagatactgatccctctgttccacctaagaccaattaaattacaagcagaatccaggcttctgagcattttaaaatttcccccaagggatcatgtacaatcagggttgagatccactggtggaggtgagctccacagccctgccctccaagtatgattcttgatgagtggccttggcatcagcacaacgtaggaacttcccagtaacacacagtctcgggctccaccttgacctactgaatcagaatccacattataacaagatcccttggtgatgcatgaacacattaaagttggggaaatggggttctacaggaaggaatggatgaatattttcacaggttcctcttctcctactacacaccaggcactgggtgggctatacttaagtcacttaaacttgcctgtgtaggttttctactgctgtcctgacagattaacataaacttagtaacttaaagcaacactcatttattttctcacagttctgtggattggcagtctggggaggctcaagtgggttctctgctcaggatctcacaggcccagagcagggtattgctgtgttaggttcttaactcaggcttggggaaggaatccacttctaagctcaattacgtttttggcagaatcaagcttcttgcagttgtaggactgaggttgctgttttcttgtgagctgttggccaggggttgccttctgcttctagatgtctctttgagttccttttaacttttacattatgttcaaagatagcaaccattcatcatatcctcctcatgcttccaacctctctgactcctccttccgctactagctagtgaaaacttgcttttaaagagctcgtgtgattatattaaactcacctccataatcgccaattttactaattcaaggttgatggattagtaaccttaataacatctgtaaaattcctttttccataaatgtgttatctcgtatattcccagtcactggcattagggctgaaggtcttgggggacatttaagaattctgtctacctcaatgtaccatgccacttacacgtcagtcttagagtcagattttgaatctaggtgtgtctgatcctaaggcttatatgaacattattttaccaatttgtttctctgtggtaagaacaaaggtgttctttgttcagagaaatttatagttatcaaagagctttcacatttattttattgtttggtctcataaaagacctttattaggtattattattctttttatgggggattgagaatgtttaattatttgttcaagggcctataagcagaatatagaaaattcaggactgaagaatgggtctcctgattccaaatttcatacttttccttttatattaccacaattttataatttcttatttagatcattcttgttgtctaattagaaaacaaatttaccaggatagaataaaagaaactagcagagtagttgtagataggatgcaaatgtctgaatcctgcagtgggccctgcacagaaaaatagacccacctgttacgctaattgaaggaaaaactctgctgaaattcagagaagtactccattcaggtcttaaaaattattgttcttaaagaagacagtcattcaatttttaaatgtaatttagaaaacaaccaattcacaaaacaaacactttttactgaattacaagtcaatcatgaccttactttggagaaatgacaggaaatattggcaaatcatgtggatgcaactcacatttgtgataagaaagttagcctgctcccatggatgaagcttaaggagaatcataaaaccatcctccttctagtgactatctttcagttcattctctttttgtttcaaaagcaaagaaaccaatgtgacctgaatgaactataattacaaagctaagattctttcagagggcaggatgatatctactggttggggttttcttggcatggccaactaggattctggtatatagggcatgtctctcatgagtcccctaataatgtaatcattttttcttctccatatggtgcaaaagtcatatctagtgagaaagtatccttacattgccagtttagaagttattttatgcttaaaaaatggcccagtcagttgttcaaataaaaaacagctggaaattcaatatcttgggctgtttccttgtcatcatttatagatgtaaggggtttcattacaatctgagaggcagtctatgatttaaacaaattatcaaaaaaattaggccttggtcagctcaattttattaaaagccttcagatcttaaaggatcaatgactacaagagaaaggttaacccccagggctcctggttggtgaacaaacacatcaaagtgaaatcagagttaaaagctattgttcccttggctaacttttgcctctgtcatattcagttgatttgaagagatgaggaatgataaacaggaccaggttacaaacatagaactgttacattttgttcatttagccaggagctttattcttttgtttttcatgagatgggtcattttaatagtcaacggtgttgacgacagtcaccattcaatctgtcatttctaatacagtctttcctaggagaatatttctcacgtgtttgacagaaaacattatctgtccatcatttccatggattcctgggtctcacgggcagaaggacaaggcagatatgaggcggatctggtaaagtaagtcattgtgtactctttgtatttgtttgaagatatttggtctttttcagtcatatatgtgatggagaaccagttgttagaacaatgtgtatattgatggagaaacaggtgggccagagtggtcggtagtctgtgtgacaaacagtgatgccactttcactatctgaaaatgaatgaatatattcatagtagtgggcatgcaaaggtaataaagacctgacccccaacatcaataatataataatgatgaattcatattctaaatctgatcatttaaggaaggccatccatatctccatcacaatcacttaaacaaatgcaaaaatggatattctttctagaatatttctgatgaaattgcttctgaaggctgcaaattagtgctcaagaccctgttgaaaagcagtttcctgtattcacttatgaagtcaaatgcagaaattatatttatttggattttatttatagcagagagaataacttaaaaactgacatagcattcttttcaaatctgaactcaatgtctgatttttggaagattcatatcagctctactcttataaatcagaaaacaaaaacaaaacaaacaaacaaaaaacaacaacaaaaaaagaaaaacaggcccagacaccagcagtgacccagtcaaccactggccagtcaatatgagagccagctggttcttctagtgaaaccttcacctttctaatcagagggtttcaggttttgctctctattgagtcaattgcttgagggtagaaaaagaaaatcttcgaattgcattacataccactcctttccctttctatagatttccccctctctcctttccaggaatattgattttcttccctgggtttctgaaaaagcttttctccccaggcatctttatttggtttgctgaccaaagcattattcacacttctcctgcggccacgccaatgccacacccgctgcaaggtgctcccggtctcctacctctgaacaacagtggtctgaatctctgacttgagccgtgcagccctttgaaagaaaagtcatttaggagctcagccctctgaggatgtaaagcccgtcgcaggtgcttgttttgtctgtctccgtgtgtggaagatgccttctgtgaggtcctgcgcctctccgtaagcagctgagtagttccttgggctgacaaaatactttgttgtggctccattacacacccagggcaacctctttagctggattttgcagaccgggaaatgggctctgaggggaagtcacgcctcatctcaaggtttactgaggagccacgaggaggccccaccgctgccacagctaactcatggcctccggccaggaagtctggagattttaagaccataatgtcagccagggtgacctctggaacctgttcaccccttcacccgttgtgaacaagagagctgaatagccactatcacagataataacaacagctgacattattaataggatgccttacaggctgtaaaatactttcacaaacaggatctcatttgatcctcataatctcaacatgaggtgcgtaaagcaagcaattattactaatctccttttacagaagagaaaaggaagtcctgagagatgaatccacttctgggaggtctgacaacgttcagctttacctaagccatggtcaggaaacttttctgcgttccaggaaatggccggccacaacgactggcccttccctataaaaacttacaaaaccctcacaggtgacctccttgtttacctatgacagaaccagacacagtgccagatcctccaaactcccattctttgccttatatgtaatcagttgaactgtttgtatctactgactaatctagacaaggtacttgctaacttgacctgtttaaaagttcgaaatgccaaactttctttcttttttttttttttcccatcccaccccacccagatggagtttcactcttgtcacccaggctggagtgagtgcagtggtgccatctgggctcagtgcaacctctgcctcccgggttcaagcaattctcctgcctcagcctctagaatagctgggattacaggcatgtgccaccacacccggctaattttgtttgtttagtagagacagggtttcatcatgttggccaggcttgttacaaactcctgacctgaggtgatctgctgcctcagcctcccacagtgctgggattacaagtgtgagccacagtgcctggcccgaaatgctaaactttcatcaagatattgcaatagtcttttctaagaaagctcttccttacttaacttgtgcctggccccaaatgctaaactttcatcaaatattgcaatagtcttttctaagaaagctcttccttacttaacttgggatttgttttatctgacacagggcacagggtaaagatcagaggtggcttcctgtcactcatccagccagccacccagctatggttacccacagggcctgatagccatccctgccagcggtcagggttgcattgtggcccccactccaggccttgcttattgcaggcttggttcccatggctgctctctgtgttcttgcaaccttgcatcctgccagaatctctggaagaaagctctttggcgagaaatgaagaacaatcccaaaggtgctccaggaaagttcattattttgtgtactctggtgtcttaccttaatcagagaacagttgtctgtgatcctcaaagagggaattaaagggaggaatggaaccagaattcagtgacaactggaatgagtgactgaggtgtagcgtcaatcatcaaggtttattaaactacttagggtgcgtctggaaaaaacatgagccacaaatacatctggggttgtttttccaaagaggtttttgggagatttagtatttatacatttccttagagggaaaaggcatgtggaaagaggggcaggtaggcagttggcaaatactacattttacataagataaggcaaatgaagagagaaagagagtaaaggaatagtccattttacttatgtctttgttctgcacctgggaggaagttcttcatgacatcagtgtggaatcaacaaactttagttttaggagctaggcttagtttgtagacctacagttataactggtggttctgttgatgggatgccagtgaagaatgtacttaggaatgatctgtgaggactgtcctttcctgatgcctgagtcctttttcttggggtgagcggggggtacaaaataggagcatatatttatggagtacatgagatgttttgatacgggcatgcaatgtgtaataatcatgtcatggacaatgaggtatccatcccctcaagcatttatcctttcttttatgaacaatctgattacacttttttacttattttaaaatgaacaattaagttattattgactataatcaccttattgccaatgtttgtcattctgtgcctggcttatttcacttgatagaatgttcaccagttccatccatgttgctgcaaatgtcaggatctcattctcttttaagactgaatagtgctccattgtgtatatgtagcacattttctttatccattcatgtgttgatggacacaggttgcttccaaatcttagctattgtgaacagggctgcaacaaacatgagagtgcagaaatctcttgcatatactgatttcctttgttttgggtgtatacccaacagtgggattgctggaccatatggtagctctatttttagttttttgaggaactttcaaactgttctccattgtggttgtactaatttatattccaactaacagtgtaggagtgttccctttcctccacatcctcgccagcatttgttactgcctgtcttttggatataagccattttaactggggtgagatgatatctcatggtagttttgttttgcatttctctgatgatcaatgatgttgagcacttttttgtatgcctgtttgccatttgcatgtcttcttctgagaaacctctattcaaatcttatgtccagttttttgatcagattattagactttttcctatagagttgtttgagttctttatatatggcgcttataaatcccttgtcagatcggtagtttgcaaatattttctcccattatgtaggttgcctcctcactttgttgattgtttcctttgctgtgcagaaggtttttaccttaatgtaatcccatttgtccacttctgctttggttgccttgcttgctgggtattactcaagaaatttttacccaaaccaatgtcctggagagttttttctatgttttcttgtagtaatttcatagtttgaggtcttagatttaagtctttaattcattttgatttaatttttgtatatgaccagagataggggtctagttttttcctgcatatgaatatccagtttccccagaaccatttattgaagaaactgtcttttccccagtgtatgttcttggcacctttattgaaaattcacatattgtaggtgtgtggatttatttctgtgttttctattctgtttcattggtctatgtgtctgttttaatgccagtaccatgctattttggttactatggttctgcagtataatttgaagtcaggtaatgtgattcttccagttttgttctatttgcttaggacagctttggctattctgggtgttttgtggttccacataaattttaggattgttttttctatttctctaaagaagttcagtggtattttgacaggtattgcattgaatctgtagattgatttgggtagtatggacagtttaataatattgattcttccaatttatgaacatggaatatctttccgtttttttggtgttgtcttcagtttctttcatcagtgttttgttgtttcattatagagatctgttgcttctttaggttaattcctaggtttttaattttacttttggcttttgtaaatgggatttacaaaaatttctttttcaggttgttcactgttggtatacaggaatgctaatgatttctgtacgttgattttatatcctgcaactttactaaatttgtttatcagttttaatagttttttggtggagtctttaggtttttccaaatataagatcatatcatttgcaaacaaggagaatttcacttctttctttccaatttggatgccatttatttctttcttctgattgctttagctaggaattccagtagtatgttggataatactagtgaaagtgggcatccttgtcatggtcatgttccatatcttagaaaaaagctttcagtttttccccattcaatatgatacaagctgtgggtctgtcatatatggcttttattatgttgaggtgtgtttcttctacacccagtttttttagggtttcttatcatgaaatgatgttgaattttattgaatgcttttttggcatcaattcaaaagatccttatatcctttattctgttttatcctttatcctttattctgttgacatgatgtatcatgttgattaatatacatatgttgaaaaattcttgcctcccagggataaatcccacttggttatgatgaatgatctttctaatgtgttgttgaattcagtttgctagtattttgttgaggacttaaaggccagagattttggcctgtggttttctttttttgagtgtctttgtctggttttgcattatagaatgaatttggaagtattcacttctcctctatttttcaaaatggtttgagtaggattagtattagttcttccttaaatgtttggtagaattcagcagtaaagccattgggtcctgggcttttctttactgagagaatttttatttgatctcattacttgttattggtttgtttaggttttgaatttcttactggcacaagcttggtaggttttatgtgtctagaaatttgtccatttcttggagaaattccaatttattggcctatagttgcttatagtagccactaatgatcctttgaatttttgcagtatcagttgtgaagtctcctatttcatttctgattttatgtttttgtacctctattttttaaattagtttgactaaaaggtttgtcaattgtgtttaactataaaaagaacctttttgttttattgatcctttttattattttttttcatttcaatttcacttatttctgctctgatctttattacttttcttttactaattttgagtttggtgtgctcttgtttttctatttctttaagatgcatcattagatcacttatttgaaggatttccccttttttgatgtaagcatttgtagatataaacttcatcttagtactgcttttgctgtatcccataggttttggtatgttgtttccattaacatctgtttcaagacatttttcaatttccctcttaatttctccattgatccactagtcattcaggagcatattgcttaatttccatgtgtttgtgtacttcccaaaattcctcatgttattgatttctagttttattccattgtggtcagagaagatgcttggaattattttaattttttgaatgttttaagatttgtttttcacctaatgtatggtctacgcttgagaatgatccttgcactgaggaaaagaatgtatattctgcagccattggatgaaatgttctataaatatctattagatccatttggcctatagtgaagattaagtcggatgattcttggttgattttctgtctaaaagatctgtccaatgctgaaagtggggtgttgaagtctccagctattctcgtattagagtctatctttctctttagctctgacatttgccttatacatctggatgctccagtgttggggacatatatatctaaaattgttattcatatattatcttgctgaattggccctttaatcattatatagtgaccttgtttgtcatttcttatagattttgtctcaaaaatctattttgtctgaaaatatagtgactcctgcttatatcagacaaatttgatatttttccatccctttattttcagtctgtgtgtgtctttataggtggtgtgtttcctataggcaagatatcagcaggtcttgcttttttcattcatttagccaggctatgccttttaatttgggagtttagtccatttatattcaatgttattattgataagtaaagacttcctcctgccattttgttattgttttctggttgttttgtggtcttctcttccttctctctttttcttcctgtattcaattaactgaaggtgattttctctggtgatatgatttagtttcttgcttttccttttttgtgtatccattgtatgttttttggtttgaagttaccatgaggcctgcaaatactagcttataacccgtgattgtaacccaatagcaacttaaccactgtttgcataaataaacaagcaaaaagataactaataaacactctacacatttttttttttttttgagacagtgtctttgctctgttgcccaggctggagtgcagtggtgcaatctcagctcacggctctttctgcctccatattcaagtgattctcatacttcagtctcccaagtagtggagattatagtcatgtgccagcatgcccagctgatttttgtgtttttagtagagatggggtttcaccatattggccagtctggtctcgaactcctgacctcaagtgatccgcctgcctcagcctcccaaagtgctgggtttataggcataagccacaatacctggccaacattctacatcttaacttcatccccccactttttaacgttttgttttatctatttacattttcttatactgtctatgtcttgaaaagttgttctagttactatttttgactggttcatcatttagtctttctacttagaataaaagtagtttacacaccacagttacagtgttgtaatagtctgtgtttgtatacttaccattaacagtgagttttgtatcttcaggtgattacttattgttcattaacacccttttctttctgattgaagtactccctttagcatttcttgtaggacaggtctagtgttgatgaaatcctcagcttttgtttgtctgggaaagtctttatttctctttcatgtttgaggggtattttttgccagatatactgttctggggtgtacattttcttctttcagcactttaaatatgtcatgctactctctcctggcctgtaagatttccattgaaaagtctgctgccagaagcattggtgcttcgttgtatgttaattgttccttttctcttgttgcttttaggatcctttatccttgatctttatcctgaatttgattattaaatgccttgaagtggtcttcttcgggttaaatctgcttggtgttctataactttcttgtacttggatattgatatctctctctaggtttgggaaattctctgatatccctttaaataaactttctgcccctatgtctttctctgcctcttctttaaggtcaataactctcagatgttcccttttgaggctattttataaatcctgtaggtgtgcttaattgtattttattcttttttcttttgtctcctctggctgtgtattttcaaacagcctatcttcaggctcactaattctttcttctgcttgatcagttctgctattaaaagactctgatgcattcttcagtatgccagttgcatttttcagctccagaatttctgcttgattctttttaattacttcagtctctgttaaatttccctgatagaattctgaattccttctctgtgttatcttgaatttctttgagtttcctcaatatagctattttgaattctctgtctaaaaggtcacatatctctgtttcattaggattggtccctggtgccttatttagttcatttgataaggtcatgatttcctggatggtgctgatgctagatgttcttcggtgtctgggcattgaagagttaggtatttattgttgtcttcactgtctgggcttgtttgtacccatccttcttgggaaggctccagatacttaaagaactagcgtgttgtgatataagctgtatctgctttagggggcacccaagcccagtaacactgtggttcttgcagactagcagagatataccatctggtatctcttggtattgatggtcgtggacaagatcgaggagaattctctagattaccaggcagagactcttgttctcttcccttacttcctcccaaacaaacagggtctctctatctctgttctgagccacctaaagctggaggtgaagtgacacaagcacccctgtggctaccatcattatgacggcacttggttgaactgaagccagcacagcactgggtctcacccaaggtctgctgtaacctctctctggccactgcctatgttcactcaaggcccttgggctttagagtaagcagatggcaaagccaaccaggcctttgtcttttccttcagggcagcaagtttgcccaggcccctggagggtctagaggtgccatctgggagtcagggactacagtcaaaaaccttagaagtctacttggtgttctactgtattgcagctgagctggcactcaaaccacaagacacagtccttcctgctcttccttcccctttccaaaggcaaaggagcctcaccctgaagtccctgccaccacaggtcacagggagtactgccagactactgccgatgatcccttaagacccaagagctcttcagtcagcttgtggtgaatgctgcctggcctgggactcacccttcagggtagtgggctcccttctggacacaggcaggtccagaaatgccatccaagagtcaagttctggaataagggaccccaggagcccacttggtgctctacccttctgtggccaaaccagcacctaaggtgaaggacaaagtcccctttacttttccttctgcttttctcaagcagaaggactctcttactagagctaccatagctgggaatgtgccgagtctcacctgaagccagcaagtctcagaggctcaccaaggccctcaacatagttcctgggtattgctgctgtttattcagggcccacgggctcttcagttagaaggtgttgagtgctggcaggactgagttcttcccttcaagacagcaggttcccttctggcccgggatgtgtctagaaatgtcatccaggcgccaggtcctggatcaaagccctcacaactgtgactggtatcctatcctgctgtggcttagccggtatccaagatacaagacaaagtcctccccacccttccctctcctctcctcaagcagaaggaaggggtctcttttggagccacaagctgtgcagcctggggttaggggaggggcgatgccagtactcccttgtcttccccagcttgtgtctcagtatgtcgcccatccccagtccactgtctctgggcctggttcagcagtagctcttgcctaagagttgcagttcctgtggcctagactgcttttcaagtttacttggagatacagagcgctgtagccctcagtggtgaggtttgcagaaactcaagtttgcacggctgggatctgtgatcctttctggctagggctggtttaaatgttccctctgtgggtgagagtgagctgagttaggtcctttcggttttcctttctgctctaacaggacagcactgagttcagtgcttcacaattgctgtgctctccctcctctagtgcctagagatgctctccacaccacatcacaacggtttttcctgcctctgaagttaaaaccaggtactatgagggctcacctgatttttggttctgatgaaggttgtgtgtgtgtgtgtgtgtgtgtgtgtgtgtgtgtgtgtgtgtgtaaattggtgtccttgaagggaggatgatgggtggagtcttctattttgccatcttgctccacctccacctcacctgaggccttttacctctctctgaggacccgcctaatgcgtaatgctggtaacaggtattcatttgggagaaggtgttgcagtgatcttcccttttgcataagaattttggaggggtcctgagatactttaattaattgaagaataatcccaaatgttctccaggaaagtttatgttgttttgtttatgctggtggtttaccttaacccagaaaagttgctgtgatccaaaaaggagcaagttaaagggaggaatgaaacaggaattcaggatgaaaaaatgagaaatctttccaatggttgttgttttgtttatgatgaatgccacggatatcagacattcttatgcagaagtgagtttaaaagatccaaagcatttccaccgttttctgtttaaagagcagcaacaagaatcacacatgttccaacatgcagtttagagaggctagaggcacagatatggacagacgtccctgctcctaacagctctctaaggtctggtggaggattcagacacatgacctggcctggaggattgagcttctggattgtctgtaagctaggcaatccactatttagtctttagtactgtaatagaggtctcagtaagtgtgtaccttgtttgcctactttatatatttttattttgtgcgataccaaatattgtggaaggatttcaggtaggaattttgagtgttgtttttgcatcaatttataaagatgacggtctctgagctttgcaggcagtatgtctataccgtgttgattcatgtgcctggctacaggtcaccacacactatacactcttgagtttgctctggagaaatctcaatgagccacctgcaacataacctgctttgtggctgggttccttaaaatccaatatattctgaaggatgtgatcaataagcagatggctcaagcccatacacatgccaagaaatgaggcatctaattaacagttagacaagggtgtgagggaattgcagaggggtgtggaggccctgcctgggctgggagacctcgggatgggagaatcagggctggttgtgtgacgtgtcgacacatagtggctgttggaagtgtgaacacagtcgggaccttcaggctgtgctcattagggctttgcaaaattcccaattatctcttgacctggccctaagcaaggcccctttccattgccctggaaaaaaaaaatgagtgagtcaaaaaggacacctgatttgacacgctacatgggtttggttctgaagctaggctagtagaacacagaaatgaggcattcttgtgcaaccagtgatgactacaggaaggataagtaccaggagcatccggtgtcacagaggcaagggcgggctttttgagatggctgtatggtgccccaaacaaaggccagaaagagacgatttgtgagaagagaccaacgcgccccttgcaaagaattcataagcagtgtttcagttaaactgcaaatctcatggatggtgtcaaaagagtgaggactcctttccgtacacgtctcacagctcaaacaggaacagaaagaggctttctctctgtgtcttggagaacccaccactaagtgctccctggtgtcagagaagggaattgggctcagtgtgacagctttccctgctatatgtgaaatacattatcaatctgttgtcagcctgatgctccctagctgactgttttgttgttgcgcttccagtgttaccctgggttggtccctgcgtgatgtttctaatataaaatatgcagattgtgaaagagaagacaatgcttcgagtctgatctatcctaagatgaatgtgctaatgctcccaagacccataagacagaggaggtcaagaaggtgccttgtggtaggcgatgcatcttcaaattcgttgacacaggctcgtgaattcagattagcacttgaccacaaatacacatgttaaaacaaagtcacattaaacatctctcttcctcaatctcctttcccagcttccttgcagagaagaaatgcaagaaggtgagtgaataaaatcagaattatttgctttttattctgaggacaaaagacaactggttggattccatgggcacacagtgatctaaggttatagtaaccaacaactatgactaagaaagtgatagtcattgtgatagttaattttacatgtccatttggctaggctatggtgcccaattgttttatcaaatgctagctggatgttgctgtgaaggtgattaacatttaaatccataagctttgagtaaagttgattaccgtccataatgtgagtggccctcatccagttagctgaaggacttacgagaatgattgaggtttctggaagaagaaattctgcctcaagacttttaacatagagactctcagcctgcagattttggactcaagactgcaacatcatcttgtgcctgaaattccagtaggctgccttgccctacagattttggacttgtcatcatcccccataatgacatgagtcaattccttaacataaatctctcctatatatcctactggctctgtttttctggataaccctgattaacacaatcattctgtctattgtagatgatctgtcctccttgaccacactcattggccaacactagccttattacctgcaaacatgagatagcatgatctattgcccagaaaagaggatagaatagaggctatttttttcctcccatctccctgttcccctgtcctctatccttatcttaatctttccaacctactattatgctccaagagtgttacctacttttattattttctgtcttcaaagttaaagagtgcctgaaagtatgcagataattcaaacaaaaaagcaacacttccctgtgtaattattcgctcaactctttgccttggtgtaatttatgtgctcaacacttttccttggaatcttagctaaagaagacttttctggggactgggcgtggtggctgaagcctgtaatcccagcactttgggaggccgaggtgggcggatcacgaggtcaggagatcaagaccatcctggctaacacggtgaaaccccatctctactaaaaatacaaaaaaattagccaggtgtggtggcggacacctgtagtcccagctattcaggaggctgaggcaggagaatggcgtgaacccaggaggcagaacttgcagtgagccaagatcgcatcattgcactccagcctgggcgacagagcaagactctgtctcaaaaaaaaaaaaaaaaagaacacttctggaaactgtttttcctggcagtccttggtcaagttgctaatttaatattttagatggttttgacatggtttagaatgcaaaattatcatcttttaatatgtatttgtttgcagagaacccatgggccttagttcatttctgcacccacagagaggtttaatctcatttaaatgctaaacatcgcagtggtcaggcattaggaacactgctaggaaggctgcaacaaaacaagtgtttccacttagtgttatttgggggttaccatccacatcatacaggaaatggagtgacaaataccaatttgagaaaggaacacaatgaaactacataattcctcttgtaggttagttgatctgtaaccaagccttaaaaattgacattgacattgaaccactgcctgtgaagggagaatgagaaataacctcaaatctgcctctaaataaaccatccatagcttaattcaagagttgggataccagctctctagcattcaaatggaatttaggtatttactaggcatactgtgggggatttttaagttgaatgggtaacatagagcattggggcaaaataatagaatacggttgctggtttcaatgacagcatgggtcttttccaccaagagactacagtacaaaatttaaatcaggtaaactggtccaatgtagaaagcaggcagtcagggaagcatagtttaagggtggcattgaaatagttttgccacttcaatttggtcactagcttttgggatcagagtatagtgtcaatgaagagagtcaaattctgtaaaatatttgaagagatttattctgagccaaatatgagtgaccatggctcatgacagccctcaggagaccctgagaacatgtacccaaggtagttggggcacagcttggttttatacactttagggagacacaagacatcaatcaaatacatttaagatatacattggttcgattcagaaaggtggtacaacctgaagtggcaggggggtggtggcggggcagcttccaagttataggtagatttaaacattttctgattggcaattggttgaaagacttactatcaatagaaagaaatgtctgagttatgataaaatgttgctgagaccaaagttttatcatgcagatgaagcctccaggtagcaggctctagagagaatagattgtaaatatttcttatcagacttaaggtctgtgttgatgttacatgctggtcagctcttcctgaattccaaaagggaggtggtataacgaggtatgtctaacctctctaagagctccctcttagaaacaaacagacaaaacacacaacaaaaaccacacttgtaaacccatcgtcccatctctccacagcttgacttcttttcataatccagatttggcttagggatccaagagtcttgaaaatatttcccatgcatttattctgaaatttgccaagggtaatttgactcctccctttgggttttgtgtttatggtgcctgagatttcaaatttgacattgttaattttgttccccacctccaatcagccttgcccacctcaacaaatgtccacttcattctttcggtgggggtcactctggactttgttctttctctcaaattgtcagtcaacaactctgtcggccctgcctttgaaataaattcatctaggatcctgcccctcttcaccactgccaccaccatgctggctaaagccactgttatttctcgtaggttaggacaacaccttctgtctggtgttgcctctactgtctagtctccacacatagccagaatactcttaaaacatacatcagataccatcatttcttagcttgccattctctaatgatgtcccacaattcttagagtaacatctcaaaatgtgaccatgccctgtgtattagtcgtcctcatcctcctcctcctcctccccttcttcttcttcttcttctttatcatcattaaactttaagttctgggatagatgtgcagaatatgcaggtttattacataggtatacatgtgccatgtggttttctgcacccgtcaacccattgtctaggatttgagtgctgcatgcattaggtatttgtcctaatgctctccctccccttgtcccccatcccctgagaggccccagtgtgtgatgttcccttctctgtgtccatgtgttctcattgttcaactctcacttatgagtgaaaacatgtggtgtttggttttctgttcctgtgttagtttgctgagaataatggtttccagattcatccatgtccctgcaaaggacatgaattcattcttttttatggctgcatagtattccatggtgtatatgtgccatattttctatatccagtctatcattgatgggcatttgggttggttccaagcctttgcgattgtgaatagcactgcaataaacatacatgtgcatgtatctttacagtagaatgatttatcatcctttgggtgtttatacccagtaatgggattgttgggtcaaatggtatttctggttctagatcttgaggaatcgccacactgtcttccacaatggctgaactaatttacactgacacagtgtaaaagctttcctatttctcgacatcctctccagcatctgttgtttcctgactttttaatatttgccattctaactggcatgagatggtatctcactgcggttttgatttgcatttctctaacgaccagtgatgagctttttttttcatgtttgtaggctgcataaatgccttctttagagaagtgtctgttcatatccttcacccactttttgatggggttgtttttttcttgtaaatttgtttaagttccttgtagattctggatgttagacctttgtcagatggagagattgcaaaaaatttctcccattctgtaggttgcctgttcactctgatgatagtttcttttactatgcagaagctccttagtttaagtagatcccatctgtcaattttggcttttgttgccattgcttttggtgtttttgtcatgaagtctttgcccatgcctatgtcctgaggggtattgcctaggttttcttctagggtttttatggttttaggttttatgtttaaatctttaggcaatcttgtgttaatttttgtataaggtgtaaggaaggggtccagtttcagttttctgcatatgcttagccagtgtccccagcaccacttattaaatagggaatcctctccccattgcttatttttgtcaggtttgttgaagatcagatggttgtagatgtgtggtgttatttctgtggcctttgttctgttccattggtctatatatctgttttggtaccagtaccatgctgttttggttgctgtagccttgtagtatagtttgaagccagggagtgtgatgcctccagctttgttctttttgcttaggattgtcatggctatacaggctcttttctggttccacataaaatttaaagtagttttttctagttctgtgaagaaaatcaatggtagcttgatgggaatagcactgaatctataaattactttgggcagtatggccattttcacaatatcgattcttcctatccatgaggatggaatgtttttccatttgtttgtgtcctctcttatttccttgagcagtggtttgtagttcttgaagaggttcttcgcgtcccttgtaagttgtattcctaggtattttatttcctttgtagcaattgtgaatgagagttcactcatgatttggctctcttttcatctgttattggtgtttaggaatgcttgtgggttttgcacattgattttgtatcctgagactttgctgaaggttcttatcagcttaaggagattttgggcagagatgatggggttttctaaatatataatcacatcatctggaaatagacaatttgacttcccctcttcctatctgaatactctttctttctcttgcctgattgccctagccagaacttccaatactatgttgaataggagtggtgagagagggcatccttgtcttgtgccagttttcaaagggaatgcttccagcttttgcccattcagtatgatattggctgtgggtttgtcataaataggcctcattattttgacatatgttccataaatccctagtttattgagtgtttttagcatgaagggatgttgaattttattgaaggccttttctgcatctattgagataatcatgtggtttttgtcattggttctgtttatgtgatggattatgtttattgatttgcatatgtttgaaccagctttgtatcccagggatgaagccgacttgatcgtggtggataagccttttgatgtgctcttggattcgctttgccagtattttattgaggattttcgcagcgatgttcatcagggatattggcttgaaattttatttttttgttgtgtctctgctaggttttggtatcaggatgatgctggccttataaaattagggaggattccctcttttcctattgtttggagtagcttcaggaggaatggaaccaactcctctttgtacctctggtagaatttggctgtgaatccatctggtcctgggctttttttggttcgtaggctattaattactgcctcaatttcagaacttgttattagtgtatatggggattcaacttcttcctgggttagtcttgggagggtgtatgtatccaagaatttatccatttcttctacattttctagtttacttgcatagaggttttcatagcagtctctgatggtagtttttatttctgtgggatcagtggtgatattccctttatcatttttttattgtgtctatttgattcttctctcttttcttctttattagtctggctagcagtctatctattttgttaatcttttcaaaaaaccagctcctggattcattgattttttgaagggtttttcatgtctctgtctccttcagttctgctgttagtgtgttggttttagatctttcctgctttctgatgtgggcattatagtgctataaatttccctcttaacactgctttagctgtgtcccacagattctggcatgttgtgtctttattctcattggtttcaaagaacttatttatttctgcctcaattttgttatttacccagtagtcattcaggagcaggttgttcagtttccatgtagttgtgtggttttgaatgagtttcttaatcctgagttctaatttgattgcactatggtctgagagactgtttgttacgatttccattcttttgcaattgctgaggagtgttttactttcaattacgtggtcaattttagaataactgctacgtggtgaagagaagaatgtatattctattgatttggggtagagagttctgtagatgtctattaggtctgcttggtccagagctgagtttaagtcctgaatatccttgttaattttctgtctcattgttctgcctaatactgacagtggggtgttaaagtctcctactattattgtgttggagactaagtctctttgtaggtctctaagaacttgctttatgaatctgggtgctcccgtactgggtacatatatatttaggaaagttagctcttcttgttgcattgatccctttaccattatgtaatgcccttctttgtctttttttcatctttgttggtttaaagtctgttttatcagagactaggattgcaacacctgctgtttttatttatttatttatttatttatttttatttttttagctttccatttgcttggtaactattcctccatctctttattttgagcgtatgtgtgtctttgcatgtgagttgggtctcctaaatacagcacaccaatgggtcttgactctatccaatttgccagtctgtgtcttttaattggggcatttagtccatttacttaaaggtaatatcattatgtgtgaatttgttcctgtcatcatgacgctagctgtttattttgcacattagttgatgcagtttcttcatagtgtcaatggtctttacatttcggtttgtttttgcagtggctggtaccagttttttctttccatgtttagtgcttccttcaggaactcttgtaaggcaggcctggtgttgacaaaatccctcagcatttgcttgtctataaaggatttttttctccttaacttatgaagcttagtttggctggatataaaattatgggtcgaaaattcttttctttaagaatgttgaatattggcccccactctcttctggcttgtagggtttctgcagagagatccactgttagtctaatgggcttccctttgtaggtaacctgacctttctctctggctgtgcttaacactttttccttgttttcaaccttggaaaatctgatgattatgtgtcttggggttgctcttctcgaggagtatctttttggtgttctctatatttcctgaatttgaatgttgacctgtcttgttaggctgtggaagttctcttggaaaatatcctgaagtatgtttcttggaaaatatcctgaagtatgtttggaaaatatcctgaagtatactttccaacttggttccgttctccccatcactttcaggtacactaatcaatcataggtcttttcacatagtcccatatttcttggaggctttatttgttccttttcattcttttttctctaatcttgtcttcacgctttatttcattaagctgatcttcaatctctgatatcctttcttctgcttgatcgatttggctattgatacttgtgtatgccttacgaagttctcatgctgtgtttttcagctccatcagatcatttatgttcttctctaaactgcttattctagttagcaattcctctaaccttttatcaaggttcttagcttccttgcattggtttagaacatgctcctttagctcagtggagtttgatattacccaccttctgaagcctacttctgtcgatttgtcaaactcattctccatccagttttgtgcccttgctggagaggagttgcaatcatttggaggagaagaggcattctgttttttggaattttcaacatttttgcactgttttttcctcatcttcgtggatttatctacctttgatttttgatactaatgacctttgggtggggtttttctgtgggcatcttttttgttgatgttgatgttattgctttctgtttgttagttttccttctaacagtcaggcccctcttctgcaggtctgctggagtttgctggaggtccactccagaccctgtttgcctgggtatcaccagtggaggctgcagaacagcaaatattgctgcctgctccttcctttagtagcttcgtcccagagtggcatctgccagaagtcagctggagctcttctgtatgaggtgtctgttgaaccctgctggaaggtgtctccctgtcaggaggcatgagggtcagggacccccttaaggagacagtctgtctcttagcagagcttggacactgtgctgggagatccgctgctctcttcagagctgacaggcagaacgtttaagtctgctgaagctggatccacagccgccccttcccccaggtgctctgtcccaggcagatgggaattttacctatcagcccctggctggggctgctgcctttctttcagagatgccctgcccagagaggaggaatctggagaggcagtctggccccaggtactttgccatgctgcggtgagttctgcagtcagagttaacactgtaaggggaaaagcacctactcaagcctcagtaatggtggacgcccctcccccaacaagctcaattgtcccaggttgacttcatactgctgtgctggcagcgagaatttcaagccagtggattttagcttgctggactttgtgggaatgggacccgctgtgcgagaagacttggcttcctggcttcagccccctttccaggggagtgagtggttctgtctcactggggttccaggcactgctggtgtatgaaaaaaaactcctgcagctgtttatctgcccagagagttgcctagttttgtgcttgaaacccagggccctggtagtgtaggcacacgagggaatctcctggtctgtgggtggcaaaaaccatggaaaaagcatagtatctgggctggatagcacagtccctcacagtagagtccctcagggcttcccttggctaggagagggaggtccatgaccccttgcacttcctgggtgaggcgataccccaccctgcttctgttccccctccatgggctgcacccactgtctaaccagtcccagtgagataaaccgggcacctcagttggaaatgcaataatcacccaccttctgcgttggtcttgctgggagctgcagactgaagctgttcctattcagccatcttgccaactctcttgtattagttttctattgctgccataacgaatagtctccatcttagcagctaaaaacaacacccatttatcaactcacagttctgcaggtcagagtctcgtaggcttggctagtttctctgtcctgagtctcatcagattgacagcaaggggctgacaaggctgtattcccttttgaaaattttggagatggatgtgtgtctttgttcattcaggttattcactgaattcagttcctgtggttgtagcaatgagatctccgtttcctttctggcggtcagcccagggtagcctttgctcctagatgctgcttgcatccctcaatctttccaggtggcccctccacccacagcaggtagggtccaggtccctctcttgctttagatctttcctccttactcttctcactccagccacatttctctcactccagccagagacatttctctaattttagatgggttccactccctggtttaaggtctgctatcttaattgcatctgccaaatctcatcatagcagtacccaggttaatatttgattgaattactgggagataggaatagtgagggactaccacagcctaggaagtcttgaatgatatgattcctgtgacttctctgacttcatgtcatccctctttcccttttaatatctagactccaagtcagtatggcctccttgctgttttctccaattgaccaaacctatatccacttgagggccttgacacctcacatttcctctgccagaacacccttgcccgaggcctttccatggcccactctctcactaagttggatgagtcctctgggaagcagactccaaggcagtattaggagagctcaagatttattgggggtaaggcctgtgaaagataaaggagagaagggacaggagtgggaaggctgggccttcagaccacagtgcaggtctgacatccttgcagggataggaggggataggaggattggatgaagagcctcagatttccatgcatactgcactgagaaagtgtcagccagcccagcagggagcttttgccacagagattgcctgtggaagggttccacgctgcccgggaaatggcaagcctttgtatcattgtgctccgtcattggctgaggattatccaggaagcatgtgacctccactcaaaagctgagggagaaacaaccaaatgtccatcaacagatgagtggatggacaaaacgtagtatgcacattcagtggaatattatccagccatgaaaaggaatgaagtattgacacacactaccacatggatgaacattgaaaacactgtgctcagtgaaataaaacagtcacaaaaggacaaatattgtatgcttctacttatggtaaatatttagaacaggtaaatccatagagacaaaatatagattagaaggtccaaggcttgcagaaggaagaaatgaggagttatcatttaacgggtacagtttctgtttgaggtgttaacaatttttgaaactggatagtggtggtgatagttgcacagaattgtgaatataattaacaccactttaaaatcttaaaaatggttgaagtggcaaattttatgctaaatacattttactacagtaaaaaacaaaacaaaacaaaaaaacagaccgaggcagatcctgaaagcaccagcagctagaagctgtcagcaaatagcaccttttgtgggaagcacatctccatggctgccatgctcactgcctcgggtctctgccgaaatggcaactgagcagtgagtcccttaatgactaaattacatccaagaggaaggcctatccttctcagtcaagttaatttttctccattacacttaaagccttctgacttatatatttacctgtttattttctgcttccccaatagaccataaacaccatgagatcagagcatccatctgtagactcacagagcaagaagcgtgactgccccaatcttgaatggatgagtaag

SEQ ID NO: 59 - RNA, 2861 nt, Homo sapiens
  source 1..2861: mol_type = unassigned RNA
ctcgcaagacctggttgtttaaaagtgggcggcaccttccccttcgctcttcctcctgctcctgccctgatgtgtctggatggtgacagatgggaatcttctccagtgaccagaatccatgccttaccttgggagcccaagctgacttctcaagctctggggatgcctcagtgatctctgatgtggaattagtggaggctggccgttgctcacctctacacagcctgctggtcgttagcgagcaggagttctgatgttcctctcatcttggatgtctttcctaggagaatatttctcacgtgtttgacagaaaacattatctgtccatcatttccatggattcctgggtctcacgggcagaaggacaaggcagatatgaggcggatctggtaaaaccataaacaccatgagatcagagcatccatctgtagactcacagagcaagaagcgtgactgccccaatcttgaatggatgagtaagatgaaaatcaatttataaacatcttgtgacaagctggaattcagttatagatcaattacagattgctcactggacaatcaaggacattattagaaaacggtttccaccactagaaattcatctacattgacatccacctaaatatccagaaggtcatccccactttcgtcgctctccacagtcagctgccgggtccaccacttcttaacttcagaaccgcaggaagccgcgtcagtcatggggttcattttgcacacgacagatttcatggttgtccttcctccaaaccgaggaacctagatcttctctgatctctgaaaaataagttcctggatatgaaaggggatactttccttggtggtagtcccagtgaagacccactgaacatcgtcagcctcaaaatgtaagctgtgctgtcatctgctttgtggaacacatatgctacacatcttctcctttcaattgggctgaagttggggcacagttaaagagcattataaagctcctgctttagcatgaacttagttatctatagaaaaaaacatgtacaaggacactgggctgtggggagcattgctctccctccattcctgagtgctcttaatgggattatcctggctttccaaaaccctatagagaagaagctcatagaagaaaattctcttactgaatcagtaaaatatggaaaataatgggactgtttattaaaggattgaatgagagaacacaagtaatgcacttagaagagtgactggcatacagtgagtactacgtgctggcttctcaaccatgatagcctgaaatgtacccggaaaatgggggctaatgtaagtcatatttagagaagttattttgggggacaatgtttttgacaagactacatttttcattatgttgctgtctgtaaacaactgtagatgcagacttgcattttgaaaggcaagacccaaaacacacaaacagagtaaatacctttaaaatgcctcgatcgctggagaaatgcctggatggacctacctgagggcagacgccactgcccaaatttcctctggggtttccctgcgtcggctgcatcttgccgacttcctcctcgatccgacagcgtggggctcaggagctgctgctggctgcttgtctgcatgggaggagaagcacacagttaccgtctttttaaccctgcgctctcctccttttactataagaaaggaaaacacatggcaggaggacaagtgggaagaacaacatggactcagagtgtccacaatggggaaaagtgaaaatgggtataaagggtcacagaagaaaaagagccaccactgcacgccctgctgaaggagacaccactcttcctgggacatcttgtcctgggtaacccccactgcttcgttcccctccatgcctgagaatgtcattgtttcccttcatatcttcgctggcaaaccagggggtaaggaaggggaactgcaggaaggaaggtggggcagtggggacgggctgggcgggggcagtctactgtcaccagcctggagatccacacttagagcttcagggaaagagttctctgcaggcaaagctgtatgatgggccctggtggaggatggagctgataacaatctaagctacagtgaaagaaagagagatgccaagacttcccacacatttcacctgttctcaggttcacctgtcacctctccctttcctaacaaaagccttggtcttcacatctctttagtatccttttttttttttttttgtcacctctttctttcttaggctttttcatctaaaaacagagggctctgaaatcatcactttccccaacctcattagccctgtctcactgtctgtcctgacttcagcctgcctccctctcccatgcgagacattgccaaccatcttcagggtgaccagtggcaaggccactgcagatgcctccccttgccccttggttgactaactccgcagaagtccctgcagtcggtggcagatgatttctaaaggctggggagcccaaaacatgagatctactgaaaactgagctatggcaccagtgggcctcctggagcaccctgctgggccgtggagccttaggcttccaaaggtactctggcccctggctgcgttgctgcacaccatggagcctggtgctgctgggggctctgcacagagcacgggatcagctccacgttgttaacctcaaatcgtaattgctgcctcataaaggggcaggtcctcccagccagctgcttctcacagcacaggactctccaggacgctgataactccttgtacttttttatatagacacatacatagagtttgaaaatgaaaatatgctgtgacttaataaatagaaactcctcaaaaaaaaaaaaaaaaa